European Patent Application EP 4 190 901 A1, published June 7, 2023. Title: Nitro compound detection element. Applicant: SUMITOMO CHEMICAL COMPANY, LIMITED. The sequence listing filed with the application follows.

SEQUENCE LISTING (109 sequences)

SEQ ID NO: 1 - protein, 420 aa, Anopheles gambiae
MARLVLHEVRYVLMAMLYISRGMATKIQNSPIDLYVYWFLTFIPIASLCVPQIIFRVKMLKQTKQIIHFYLSLQFTYLVVDTKSLIDFISVLVPITEILLTNGKMIICNVKRGKIINLINQVQVAWDECAKSEHLEIQTLITTTAKKSKIFVIIYTTSFLLICVEYSSMPLFKLIYHSAVYGKQSNYTIALPYLSRFAYSTESTTSFAWTYFFILIGVYLLALTLSGFDSLFSTLVMHIKMMFKVLKFEIEQLGLDLSAGKSHVELQAKLKQIILKHKTNLSLIEQLEDGFSFFLMAQFLTSSILVCVVLYELTMVFGWNEDTFKTVTYLPGAILQLFLFCWYAQQITEEARLVSDHIYNIPWYLADPKLQKDILTFMVKAQKPTGVTASKFYMVTLQTFQRISSTSYSYFTLLQTINQQ

SEQ ID NO: 2 - protein, 387 aa, Anopheles gambiae
MVVFDPLDDPLKVLPLPLKLLALLGVNKNPSERFRLYAIYAYLCIALFIPKLCLGYETILQCFRSIAEGMLSFNTTITFIMLPLKMDNLEDLLKNLKRFTEIVIFNEDYEQILIRLNTAIHKFTKYYFIFTNGIVFAMTSSTIAGMFYTYYAKDSEYSAAFPLIMENRLYLIDSHYNLGHCFVHQALMFFALYILLVMFTAKAGTLFGLIRFCSTVLGIIVLKIERLSQIGPVDKYTAELNEIIELHQLAIKCSRQLQNILMEILLAQFTGCVFIWCFMLYYVMISGITAEGIAVVAMLIALSTETFIFCLLGNELTLKGLEISTAMYFTNWYDQPVKLQKMVVPIIQQSQQRIGITAAKFYYIDYNRYGQSLKTAYSFYLLLKDIF

SEQ ID NO: 3 - protein, 405 aa, Anopheles gambiae
MVRLSFEETLRNTNLMLLMMGIPPCEEPYPPGVLPSLKRNAGFIASFLLLAYTTIGELIYLKQMFERDVTFLEVTFQAPCIGYCTIGVLKMVILARGRNTIAELVGLFRAKWTSAIVTGAHWAVCEDTMRPAIRVTSVTALANVVMGIAFTILPIAEMIYTHHYTGRWNRQLAFNIWWPFDVLGGVKYYWFVYPLYVVIGFTGIIIHMAFDCLFCILAAHLCMQFRILAHNFGHVVEVANGAREGDSGSTSRLRDAIRIHQELIGYEGTPLDAGVNQWRNGYMLVKFVLFMLCFLIELLMLCAYGEDIVESVRHQAVMSESRVIEAFAFKTHQSLGVIDAAYGCEWYREGSVAFHRSVLQIIHRSQQSVILTAWKIWPIQMSTFSQILQASWSYFTLLKTVYGNK

SEQ ID NO: 4 - protein, 387 aa, Anopheles gambiae
MNFLRQEQPAGMPHISIKLLRVFGVTNHSEERFRIVPVMLAYFFFIVVPKCFFGYPDLEIMIIGTAELIFQTNSFCGMFLLFLNRRKLAEFIQHARSFSQTVICASPPAVVRHLTTQHDMIHKITRIFCIVVMFAAHFYALAPFLSTLYTFYGTVRNKNATMHYTLQMEENFYGLQTRTSGTHYLIFGVVMTPTAYLCAFTGTVKTLTICNITTYCTLYFQLVQLKLRTVTQDNTFRQELKSVIKMHQDALNCASLVESITSLALLQQLLLCVLIWSSMLLYFTVSGFNVNFMNLFVLFVFDTTETFAYCYLGEKLSYESARVAHTIYESGWETQTTDIQKDLQLILVRAQSPVGITAGKFYYMNMEQFGIIVKTTYSFFVILRDQI

SEQ ID NO: 5 - protein, 406 aa, Aedes aegypti
MTQSLEFDQTFGFIAKVLQMIGYPSCLAPYPTTFASRLKSSAGFVVCFLMLTYCVFGQIINIGLLMMGHRQTDQVVEEVAIQVSSTGFCIIGLAKMYSLSYNRAILSWLIADFRVKWNAGELTDKDRSIRDGTLRPTVAITTVAALGNIIMVSAFNFQPVVEMIYGRVVTGEWVKLFLYVIWFPFNSTHGAIYYLVYLFEVYSGVIVAVGNVGFNCIFCLLTSHLSMQLKLLCSWIEDMVEVEDEKGVQSKKKLYRIVRYHQDLIRGRNALQSMFSTTLFLNFSASSVLMCMQLYLITTAGITLMVKFTLFMLCILMEIFILCYYGEEILANSSSIAAGAFNSNWYQSKVSQQNPRFGKNLIPIIQQGQRPMVLTAWKFWPITIRTFSAILQTSWSYFTLLKTVMH

SEQ ID NO: 6 - DNA, 1263 bp, Artificial Sequence
  AgOR28 WT
atggccagactggtgctgcacgaagtccgctatgtgctgatggccatgctgtacatcagcagaggcatggccaccaagatccagaacagccccatcgacctgtacgtgtactggttcctgacattcatccctatcgccagcctgtgcgtgccccagatcatcttcagagtgaagatgctgaagcagaccaagcagatcatccacttctacctgagcctgcagttcacctacctggtggtggacaccaagagcctgatcgacttcatcagcgtgctggtgcccatcaccgagatcctgctgaccaacggcaagatgattatctgcaacgtgaagcggggcaagatcatcaacctgatcaaccaggtgcaggtcgcctgggatgagtgtgccaagtctgagcacctggaaatccagacactgatcaccaccaccgccaagaaaagcaagatcttcgtgattatctacaccaccagctttctgctgatctgcgtggaatactccagcatgcccctgttcaagctgatctaccacagcgccgtgtacggcaagcagagcaactacacaatcgccctgccttacctgagcagattcgcctacagcaccgagagcaccacaagcttcgcctggacctacttcttcatcctgatcggcgtgtacctgctggccctgacactgagcggcttcgatagcctgtttagcaccctggtcatgcacatcaagatgatgttcaaggtgctgaagttcgagatcgagcagctgggcctcgatctgtctgccggcaaatctcacgtggaactccaggccaagctgaagcaaatcatcctgaagcacaagaccaacctgtctctgattgagcagctcgaggacggcttttcattcttcctgatggcccagttcctgaccagcagcatcctcgtgtgtgtggtgctgtacgagctgaccatggtgttcggctggaacgaggacaccttcaagaccgtgacatacctgcctggcgctatcctgcagctgttcctgttctgttggtacgcccagcagatcaccgaagaggccaggctggtgtccgatcacatctacaacatcccttggtatctggctgaccccaagctgcagaaggacatcctgaccttcatggtcaaggcccagaaacctaccggcgtgaccgccagcaagttctacatggtcaccctgcagaccttccagagaatcagcagcacctcctacagctacttcaccctgctgcagaccatcaaccagcagtaa

SEQ ID NO: 7 - protein, 1164 aa, Artificial Sequence
  AgOR47 WT
ATGGTGGTGTTCGACCCTCTGGACGATCCCCTGAAAGTGCTGCCTCTGCCTCTGAAACTGCTGGCCCTGCTGGGCGTGAACAAGAACCCTAGCGAGCGGTTCAGACTGTACGCCATCTACGCCTACCTGTGTATCGCCCTGTTCATCCCCAAGCTGTGCCTGGGCTACGAGACAATCCTGCAGTGCTTCCGGTCTATCGCCGAGGGCATGCTGAGCTTCAATACCACCATCACCTTCATCATGCTGCCCCTGAAGATGGACAACCTGGAAGATCTGCTGAAGAACCTGAAGCGGTTCACCGAGATCGTGATCTTCAACGAGGACTACGAGCAGATCCTGATCCGGCTGAACACCGCCATCCACAAGTTCACCAAGTACTACTTCATCTTCACCAACGGCATCGTGTTCGCCATGACCAGCTCTACAATCGCCGGCATGTTCTACACCTACTACGCCAAGGACAGCGAGTACAGCGCCGCCTTTCCTCTGATCATGGAAAACCGGCTGTACCTGATCGACAGCCACTACAACCTGGGCCACTGCTTCGTGCACCAGGCTCTGATGTTCTTTGCCCTGTACATCCTGCTCGTGATGTTCACCGCCAAGGCCGGCACACTGTTCGGCCTGATCAGATTCTGTAGCACCGTGCTGGGCATCATCGTGCTGAAGATCGAGCGGCTGTCTCAGATCGGCCCCGTGGATAAGTATACCGCCGAGCTGAACGAGATCATCGAGCTGCACCAGCTGGCCATCAAGTGCAGCAGACAGCTGCAGAACATCCTGATGGAAATCCTGCTGGCTCAGTTCACCGGCTGCGTGTTCATCTGGTGCTTCATGCTGTACTACGTGATGATCAGCGGCATCACCGCCGAGGGAATTGCCGTGGTGGCTATGCTGATTGCCCTGTCTACCGAGACTTTCATCTTCTGCCTGCTGGGAAACGAGCTGACCCTGAAAGGCCTGGAAATCAGCACCGCCATGTACTTCACAAATTGGTACGACCAGCCTGTGAAGCTCCAGAAAATGGTGGTGCCCATCATCCAGCAGTCCCAGCAGAGAATCGGAATCACAGCCGCCAAGTTCTACTACATCGACTACAACAGATACGGCCAGAGCCTGAAAACCGCCTACAGCTTCTACCTGCTGCTGAAGGACATCTTCTGA

SEQ ID NO: 8 - DNA, 1218 bp, Artificial Sequence
  AgOR6 WT
atggtacgtctaagctttgaagaaacgcttcgaaacaccaacctgatgctactgatgatgggcattccaccgtgcgaggagccgtacccgccgggcgtactgccgtcgctcaaacgcaacgcgggcttcatcgcgtccttcctgctgctcgcctacaccacgatcggtgagctgatctatctgaagcagatgttcgagcgggacgttaccttcctggaggtaacctttcaagcgccctgcatcgggtactgcaccatcggtgtgctgaagatggtcatactggcccggggaaggaacacgatcgccgagctggtcggtttgtttcgcgcaaagtggacgtcggcgattgtaaccggtgcgcattgggcggtgtgcgaggacacaatgcggcccgccattcgggtcacctcggtaacggcgctcgcgaacgtcgtgatggggatagcgttcaccatcctgccgatcgcggagatgatctacacccatcactacacgggccggtggaaccgtcagcttgccttcaacatctggtggccgttcgatgtgctgggtggcgtaaagtactactggttcgtctatccactgtacgtcgtgattgggttcacgggcatcatcatccatatggcgttcgactgtttgttctgcatactggcggcccatctctgtatgcagtttcgcatcctggcgcacaactttggccatgtggtagaggttgccaatggtgctcgtgaaggtgacagtggcagtacgagtcggctacgggatgcgatcagaatccatcaggagttgattgggtacgaaggaaccccattggatgcgggagtaaatcaatggcgtaacggatatatgctggtaaagtttgtcctcttcatgctgtgctttctgatcgagctgctgatgctgtgtgcgtacggtgaggatattgtggaatcggtaaggcaccaggcggtgatgagcgagtcgcgagtaattgaagcttttgcttttaaaacacatcagagccttggggtgattgatgccgcttacggttgcgaatggtaccgggaagggtcggtggcgttccatcgatccgtgctgcaaattatacaccgcagccagcagtccgtcatactgaccgcatggaaaatttggcccatccaaatgagtactttcagtcagatcctgcaagcttcctggtcctactttaccctcctgaagaccgtctacgggaataagtaa

SEQ ID NO: 9 - DNA, 1164 bp, Artificial Sequence
  AgOR15 WT
atgaacttcctaagacaggagcaaccggctggcatgcctcatatctccatcaagctgctccgggtatttggcgttaccaaccattcagaggaacgctttcgtatcgtgccggttatgctggcctactttttcttcatagtagtgcccaagtgcttcttcggatatcccgaccttgagataatgatcattggcaccgctgagctgattttccaaaccaactccttttgcggaatgtttctgttgtttctgaacagacgcaaactggctgagttcattcaacatgctagaagtttctcccaaacggttatctgtgcgtcacctcccgcagtggtccggcatttgacgacccagcacgacatgatccacaagataaccagaatcttctgcatcgtagtgatgtttgcagctcacttctacgcattagctccttttctttctacactttacacgttttacggtacggtacggaacaaaaacgcaaccatgcactacacgctgcaaatggaggaaaacttctacggactacagactcgcacctcgggtacgcactacctgatcttcggtgtcgtcatgacgcctaccgcgtatctctgtgcctttaccggcacggtgaagactctaaccatctgtaatattactacctactgtaccctttactttcaactggtacaactgaagctacgaaccgtcacgcaagacaacacgttccgccaggagttgaagtcggtgatcaagatgcatcaggatgcacttaactgtgcaagtctggtagaatctatcacgtcactagcgctattacagcaactgcttctatgcgtattgatctggagctcaatgctgctttacttcaccgtatcgggattcaatgtgaactttatgaaccttttcgtactgttcgtgttcgacacaacggaaacctttgcctactgttatcttggggaaaagctatcgtacgagagtgctcgtgtagcacataccatttacgaaagtgggtgggaaactcaaaccaccgacatacagaaagatcttcagctaattcttgtccgtgctcaaagtccagttggcatcactgctggaaagttttactacatgaacatggaacagtttggcattatagtaaaaactacctactcgttctttgtgatattgcgggatcagatttaa

SEQ ID NO: 10 - DNA, 1221 bp, Artificial Sequence
  AaOR4 WT
atgactcaatcccttgagtttgaccaaacctttggcttcatcgccaaggtcttgcaaatgatcggttatccaagctgtttagcaccgtacccaacgaccttcgccagtcgactcaagtccagtgccggtttcgtggtatgcttcctcatgttgacctattgcgttttcggtcagatcatcaacatcggcctgctgatgatgggtcaccgccagacggatcaggtcgtcgaagaggtcgccatccaggtcagcagcacaggcttttgcatcatcggactggcgaagatgtacagtttgtcgtacaaccgggccattctgagctggctcattgcggacttcagagtcaagtggaatgccggggaactcacagataaggaccgttccatacgggacgggacgttacgtccaacggtggccattacgactgtagcggcattagggaacatcataatggtgtcggcgttcaactttcaaccggtggtggagatgatctacggtcgggtggttaccggagaatgggtcaagctatttctgtacgtgatttggttccctttcaattcgactcacggggcgatctactatctggtgtacttgtttgaggtttattcgggagttatagtggccgttggaaacgtggggttcaactgtatcttctgtttgctgacttcacacttgtcgatgcagttaaagctgttgtgcagttggatcgaggatatggttgaagttgaggacgagaagggggtgcaatcgaagaagaagctctacaggattgtgcggtatcatcaggacttgatcagaggaaggaatgcgttacaatcaatgttcagcacaacgctgttcctgaacttctccgcaagttctgttctgatgtgcatgcagctttacctcataactaccgcaggcattactctgatggtcaagtttactcttttcatgctttgtattttgatggagattttcattctctgctactacggtgaagagattctcgctaatagttcatcgattgccgctggagcgttcaactcgaattggtaccagtcgaaggtgagccaacagaatcctcgttttggcaaaaatttgattccgattatccagcaagggcagaggcccatggttctgacggcgtggaagttttggcccataaccattcggacgttcagcgccatattgcaaacatcatggtcctattttaccttgctgaaaactgtaatgcattag

SEQ ID NO: 11 - protein, 420 aa, Artificial Sequence
  AgOR28 T25K
MARLVLHEVRYVLMAMLYISRGMAKKIQNSPIDLYVYWFLTFIPIASLCVPQIIFRVKMLKQTKQIIHFYLSLQFTYLVVDTKSLIDFISVLVPITEILLTNGKMIICNVKRGKIINLINQVQVAWDECAKSEHLEIQTLITTTAKKSKIFVIIYTTSFLLICVEYSSMPLFKLIYHSAVYGKQSNYTIALPYLSRFAYSTESTTSFAWTYFFILIGVYLLALTLSGFDSLFSTLVMHIKMMFKVLKFEIEQLGLDLSAGKSHVELQAKLKQIILKHKTNLSLIEQLEDGFSFFLMAQFLTSSILVCVVLYELTMVFGWNEDTFKTVTYLPGAILQLFLFCWYAQQITEEARLVSDHIYNIPWYLADPKLQKDILTFMVKAQKPTGVTASKFYMVTLQTFQRISSTSYSYFTLLQTINQQ

SEQ ID NO: 12 - DNA, 1263 bp, Artificial Sequence
  AgOR28 T25K
atggccagactggtgctgcacgaagtccgctatgtgctgatggccatgctgtacatcagcagaggcatggccaagaagatccagaacagccccatcgacctgtacgtgtactggttcctgacattcatccctatcgccagcctgtgcgtgccccagatcatcttcagagtgaagatgctgaagcagaccaagcagatcatccacttctacctgagcctgcagttcacctacctggtggtggacaccaagagcctgatcgacttcatcagcgtgctggtgcccatcaccgagatcctgctgaccaacggcaagatgattatctgcaacgtgaagcggggcaagatcatcaacctgatcaaccaggtgcaggtcgcctgggatgagtgtgccaagtctgagcacctggaaatccagacactgatcaccaccaccgccaagaaaagcaagatcttcgtgattatctacaccaccagctttctgctgatctgcgtggaatactccagcatgcccctgttcaagctgatctaccacagcgccgtgtacggcaagcagagcaactacacaatcgccctgccttacctgagcagattcgcctacagcaccgagagcaccacaagcttcgcctggacctacttcttcatcctgatcggcgtgtacctgctggccctgacactgagcggcttcgatagcctgtttagcaccctggtcatgcacatcaagatgatgttcaaggtgctgaagttcgagatcgagcagctgggcctcgatctgtctgccggcaaatctcacgtggaactccaggccaagctgaagcaaatcatcctgaagcacaagaccaacctgtctctgattgagcagctcgaggacggcttttcattcttcctgatggcccagttcctgaccagcagcatcctcgtgtgtgtggtgctgtacgagctgaccatggtgttcggctggaacgaggacaccttcaagaccgtgacatacctgcctggcgctatcctgcagctgttcctgttctgttggtacgcccagcagatcaccgaagaggccaggctggtgtccgatcacatctacaacatcccttggtatctggctgaccccaagctgcagaaggacatcctgaccttcatggtcaaggcccagaaacctaccggcgtgaccgccagcaagttctacatggtcaccctgcagaccttccagagaatcagcagcacctcctacagctacttcaccctgctgcagaccatcaaccagcagtaa

SEQ ID NO: 13 - DNA, 31 bp, Artificial Sequence
  Primer
cagaggcatggccaagaagatccagaacagc

SEQ ID NO: 14 - DNA, 31 bp, Artificial Sequence
  Primer
gctgttctggatcttcttggccatgcctctg

SEQ ID NO: 15 - protein, 420 aa, Artificial Sequence
  AgOR28 P31T
MARLVLHEVRYVLMAMLYISRGMATKIQNSTIDLYVYWFLTFIPIASLCVPQIIFRVKMLKQTKQIIHFYLSLQFTYLVVDTKSLIDFISVLVPITEILLTNGKMIICNVKRGKIINLINQVQVAWDECAKSEHLEIQTLITTTAKKSKIFVIIYTTSFLLICVEYSSMPLFKLIYHSAVYGKQSNYTIALPYLSRFAYSTESTTSFAWTYFFILIGVYLLALTLSGFDSLFSTLVMHIKMMFKVLKFEIEQLGLDLSAGKSHVELQAKLKQIILKHKTNLSLIEQLEDGFSFFLMAQFLTSSILVCVVLYELTMVFGWNEDTFKTVTYLPGAILQLFLFCWYAQQITEEARLVSDHIYNIPWYLADPKLQKDILTFMVKAQKPTGVTASKFYMVTLQTFQRISSTSYSYFTLLQTINQQ

SEQ ID NO: 16 - DNA, 1263 bp, Artificial Sequence
  AgOR28 P31T
atggccagactggtgctgcacgaagtccgctatgtgctgatggccatgctgtacatcagcagaggcatggccaccaagatccagaacagcaccatcgacctgtacgtgtactggttcctgacattcatccctatcgccagcctgtgcgtgccccagatcatcttcagagtgaagatgctgaagcagaccaagcagatcatccacttctacctgagcctgcagttcacctacctggtggtggacaccaagagcctgatcgacttcatcagcgtgctggtgcccatcaccgagatcctgctgaccaacggcaagatgattatctgcaacgtgaagcggggcaagatcatcaacctgatcaaccaggtgcaggtcgcctgggatgagtgtgccaagtctgagcacctggaaatccagacactgatcaccaccaccgccaagaaaagcaagatcttcgtgattatctacaccaccagctttctgctgatctgcgtggaatactccagcatgcccctgttcaagctgatctaccacagcgccgtgtacggcaagcagagcaactacacaatcgccctgccttacctgagcagattcgcctacagcaccgagagcaccacaagcttcgcctggacctacttcttcatcctgatcggcgtgtacctgctggccctgacactgagcggcttcgatagcctgtttagcaccctggtcatgcacatcaagatgatgttcaaggtgctgaagttcgagatcgagcagctgggcctcgatctgtctgccggcaaatctcacgtggaactccaggccaagctgaagcaaatcatcctgaagcacaagaccaacctgtctctgattgagcagctcgaggacggcttttcattcttcctgatggcccagttcctgaccagcagcatcctcgtgtgtgtggtgctgtacgagctgaccatggtgttcggctggaacgaggacaccttcaagaccgtgacatacctgcctggcgctatcctgcagctgttcctgttctgttggtacgcccagcagatcaccgaagaggccaggctggtgtccgatcacatctacaacatcccttggtatctggctgaccccaagctgcagaaggacatcctgaccttcatggtcaaggcccagaaacctaccggcgtgaccgccagcaagttctacatggtcaccctgcagaccttccagagaatcagcagcacctcctacagctacttcaccctgctgcagaccatcaaccagcagtaa

SEQ ID NO: 17 - DNA, 33 bp, Artificial Sequence
  Primer
cagatccagaacagcaccatcgacctgtacgtg

SEQ ID NO: 18 - DNA, 33 bp, Artificial Sequence
  Primer
cacgtacaggtcgatggtgctgttctggatctg

SEQ ID NO: 19 - protein, 420 aa, Artificial Sequence
  AgOR28 T25K, P31T
MARLVLHEVRYVLMAMLYISRGMAKKIQNSTIDLYVYWFLTFIPIASLCVPQIIFRVKMLKQTKQIIHFYLSLQFTYLVVDTKSLIDFISVLVPITEILLTNGKMIICNVKRGKIINLINQVQVAWDECAKSEHLEIQTLITTTAKKSKIFVIIYTTSFLLICVEYSSMPLFKLIYHSAVYGKQSNYTIALPYLSRFAYSTESTTSFAWTYFFILIGVYLLALTLSGFDSLFSTLVMHIKMMFKVLKFEIEQLGLDLSAGKSHVELQAKLKQIILKHKTNLSLIEQLEDGFSFFLMAQFLTSSILVCVVLYELTMVFGWNEDTFKTVTYLPGAILQLFLFCWYAQQITEEARLVSDHIYNIPWYLADPKLQKDILTFMVKAQKPTGVTASKFYMVTLQTFQRISSTSYSYFTLLQTINQQ

SEQ ID NO: 20 - DNA, 1263 bp, Artificial Sequence
  AgOR28 T25K, P31T
atggccagactggtgctgcacgaagtccgctatgtgctgatggccatgctgtacatcagcagaggcatggccaagaagatccagaacagcaccatcgacctgtacgtgtactggttcctgacattcatccctatcgccagcctgtgcgtgccccagatcatcttcagagtgaagatgctgaagcagaccaagcagatcatccacttctacctgagcctgcagttcacctacctggtggtggacaccaagagcctgatcgacttcatcagcgtgctggtgcccatcaccgagatcctgctgaccaacggcaagatgattatctgcaacgtgaagcggggcaagatcatcaacctgatcaaccaggtgcaggtcgcctgggatgagtgtgccaagtctgagcacctggaaatccagacactgatcaccaccaccgccaagaaaagcaagatcttcgtgattatctacaccaccagctttctgctgatctgcgtggaatactccagcatgcccctgttcaagctgatctaccacagcgccgtgtacggcaagcagagcaactacacaatcgccctgccttacctgagcagattcgcctacagcaccgagagcaccacaagcttcgcctggacctacttcttcatcctgatcggcgtgtacctgctggccctgacactgagcggcttcgatagcctgtttagcaccctggtcatgcacatcaagatgatgttcaaggtgctgaagttcgagatcgagcagctgggcctcgatctgtctgccggcaaatctcacgtggaactccaggccaagctgaagcaaatcatcctgaagcacaagaccaacctgtctctgattgagcagctcgaggacggcttttcattcttcctgatggcccagttcctgaccagcagcatcctcgtgtgtgtggtgctgtacgagctgaccatggtgttcggctggaacgaggacaccttcaagaccgtgacatacctgcctggcgctatcctgcagctgttcctgttctgttggtacgcccagcagatcaccgaagaggccaggctggtgtccgatcacatctacaacatcccttggtatctggctgaccccaagctgcagaaggacatcctgaccttcatggtcaaggcccagaaacctaccggcgtgaccgccagcaagttctacatggtcaccctgcagaccttccagagaatcagcagcacctcctacagctacttcaccctgctgcagaccatcaaccagcagtaa

SEQ ID NO: 21 - protein, 398 aa, Artificial Sequence
  AgOR28 22a.a del
MARLVLHEVRYVLMAMLYISRGMATKIQNSPIDLYVYWFLTFIPIASLCVPQFTYLVVDTKSLIDFISVLVPITEILLTNGKMIICNVKRGKIINLINQVQVAWDECAKSEHLEIQTLITTTAKKSKIFVIIYTTSFLLICVEYSSMPLFKLIYHSAVYGKQSNYTIALPYLSRFAYSTESTTSFAWTYFFILIGVYLLALTLSGFDSLFSTLVMHIKMMFKVLKFEIEQLGLDLSAGKSHVELQAKLKQIILKHKTNLSLIEQLEDGFSFFLMAQFLTSSILVCVVLYELTMVFGWNEDTFKTVTYLPGAILQLFLFCWYAQQITEEARLVSDHIYNIPWYLADPKLQKDILTFMVKAQKPTGVTASKFYMVTLQTFQRISSTSYSYFTLLQTINQQ

SEQ ID NO: 22 - DNA, 1197 bp, Artificial Sequence
  AgOR28 22a.a del
atggccagactggtgctgcacgaagtccgctatgtgctgatggccatgctgtacatcagcagaggcatggccaccaagatccagaacagccccatcgacctgtacgtgtactggttcctgacattcatccctatcgccagcctgtgcgtgccccagttcacctacctggtggtggacaccaagagcctgatcgacttcatcagcgtgctggtgcccatcaccgagatcctgctgaccaacggcaagatgattatctgcaacgtgaagcggggcaagatcatcaacctgatcaaccaggtgcaggtcgcctgggatgagtgtgccaagtctgagcacctggaaatccagacactgatcaccaccaccgccaagaaaagcaagatcttcgtgattatctacaccaccagctttctgctgatctgcgtggaatactccagcatgcccctgttcaagctgatctaccacagcgccgtgtacggcaagcagagcaactacacaatcgccctgccttacctgagcagattcgcctacagcaccgagagcaccacaagcttcgcctggacctacttcttcatcctgatcggcgtgtacctgctggccctgacactgagcggcttcgatagcctgtttagcaccctggtcatgcacatcaagatgatgttcaaggtgctgaagttcgagatcgagcagctgggcctcgatctgtctgccggcaaatctcacgtggaactccaggccaagctgaagcaaatcatcctgaagcacaagaccaacctgtctctgattgagcagctcgaggacggcttttcattcttcctgatggcccagttcctgaccagcagcatcctcgtgtgtgtggtgctgtacgagctgaccatggtgttcggctggaacgaggacaccttcaagaccgtgacatacctgcctggcgctatcctgcagctgttcctgttctgttggtacgcccagcagatcaccgaagaggccaggctggtgtccgatcacatctacaacatcccttggtatctggctgaccccaagctgcagaaggacatcctgaccttcatggtcaaggcccagaaacctaccggcgtgaccgccagcaagttctacatggtcaccctgcagaccttccagagaatcagcagcacctcctacagctacttcaccctgctgcagaccatcaaccagcagtaa

SEQ ID NO: 23 - DNA, 33 bp, Artificial Sequence
  Primer
taccgagctcggatcatggccagactggtgctg

SEQ ID NO: 24 - DNA, 34 bp, Artificial Sequence
  Primer
gatatctgcagaattttactgctggttgatggtc

SEQ ID NO: 25 - protein, 398 aa, Artificial Sequence
  AgOR28 T25K, 22a.a del
MARLVLHEVRYVLMAMLYISRGMAKKIQNSPIDLYVYWFLTFIPIASLCVPQFTYLVVDTKSLIDFISVLVPITEILLTNGKMIICNVKRGKIINLINQVQVAWDECAKSEHLEIQTLITTTAKKSKIFVIIYTTSFLLICVEYSSMPLFKLIYHSAVYGKQSNYTIALPYLSRFAYSTESTTSFAWTYFFILIGVYLLALTLSGFDSLFSTLVMHIKMMFKVLKFEIEQLGLDLSAGKSHVELQAKLKQIILKHKTNLSLIEQLEDGFSFFLMAQFLTSSILVCVVLYELTMVFGWNEDTFKTVTYLPGAILQLFLFCWYAQQITEEARLVSDHIYNIPWYLADPKLQKDILTFMVKAQKPTGVTASKFYMVTLQTFQRISSTSYSYFTLLQTINQQ

SEQ ID NO: 26 - DNA, 1197 bp, Artificial Sequence
  AgOR28 T25K, 22a.a del
atggccagactggtgctgcacgaagtccgctatgtgctgatggccatgctgtacatcagcagaggcatggccaagaagatccagaacagccccatcgacctgtacgtgtactggttcctgacattcatccctatcgccagcctgtgcgtgccccagttcacctacctggtggtggacaccaagagcctgatcgacttcatcagcgtgctggtgcccatcaccgagatcctgctgaccaacggcaagatgattatctgcaacgtgaagcggggcaagatcatcaacctgatcaaccaggtgcaggtcgcctgggatgagtgtgccaagtctgagcacctggaaatccagacactgatcaccaccaccgccaagaaaagcaagatcttcgtgattatctacaccaccagctttctgctgatctgcgtggaatactccagcatgcccctgttcaagctgatctaccacagcgccgtgtacggcaagcagagcaactacacaatcgccctgccttacctgagcagattcgcctacagcaccgagagcaccacaagcttcgcctggacctacttcttcatcctgatcggcgtgtacctgctggccctgacactgagcggcttcgatagcctgtttagcaccctggtcatgcacatcaagatgatgttcaaggtgctgaagttcgagatcgagcagctgggcctcgatctgtctgccggcaaatctcacgtggaactccaggccaagctgaagcaaatcatcctgaagcacaagaccaacctgtctctgattgagcagctcgaggacggcttttcattcttcctgatggcccagttcctgaccagcagcatcctcgtgtgtgtggtgctgtacgagctgaccatggtgttcggctggaacgaggacaccttcaagaccgtgacatacctgcctggcgctatcctgcagctgttcctgttctgttggtacgcccagcagatcaccgaagaggccaggctggtgtccgatcacatctacaacatcccttggtatctggctgaccccaagctgcagaaggacatcctgaccttcatggtcaaggcccagaaacctaccggcgtgaccgccagcaagttctacatggtcaccctgcagaccttccagagaatcagcagcacctcctacagctacttcaccctgctgcagaccatcaaccagcagtaa

SEQ ID NO: 27 - protein, 398 aa, Artificial Sequence
  AgOR28 P31T, 22a.a del
MARLVLHEVRYVLMAMLYISRGMATKIQNSTIDLYVYWFLTFIPIASLCVPQFTYLVVDTKSLIDFISVLVPITEILLTNGKMIICNVKRGKIINLINQVQVAWDECAKSEHLEIQTLITTTAKKSKIFVIIYTTSFLLICVEYSSMPLFKLIYHSAVYGKQSNYTIALPYLSRFAYSTESTTSFAWTYFFILIGVYLLALTLSGFDSLFSTLVMHIKMMFKVLKFEIEQLGLDLSAGKSHVELQAKLKQIILKHKTNLSLIEQLEDGFSFFLMAQFLTSSILVCVVLYELTMVFGWNEDTFKTVTYLPGAILQLFLFCWYAQQITEEARLVSDHIYNIPWYLADPKLQKDILTFMVKAQKPTGVTASKFYMVTLQTFQRISSTSYSYFTLLQTINQQ

SEQ ID NO: 28 - DNA, 1197 bp, Artificial Sequence
  AgOR28 P31T, 22a.a del
atggccagactggtgctgcacgaagtccgctatgtgctgatggccatgctgtacatcagcagaggcatggccaccaagatccagaacagcaccatcgacctgtacgtgtactggttcctgacattcatccctatcgccagcctgtgcgtgccccagttcacctacctggtggtggacaccaagagcctgatcgacttcatcagcgtgctggtgcccatcaccgagatcctgctgaccaacggcaagatgattatctgcaacgtgaagcggggcaagatcatcaacctgatcaaccaggtgcaggtcgcctgggatgagtgtgccaagtctgagcacctggaaatccagacactgatcaccaccaccgccaagaaaagcaagatcttcgtgattatctacaccaccagctttctgctgatctgcgtggaatactccagcatgcccctgttcaagctgatctaccacagcgccgtgtacggcaagcagagcaactacacaatcgccctgccttacctgagcagattcgcctacagcaccgagagcaccacaagcttcgcctggacctacttcttcatcctgatcggcgtgtacctgctggccctgacactgagcggcttcgatagcctgtttagcaccctggtcatgcacatcaagatgatgttcaaggtgctgaagttcgagatcgagcagctgggcctcgatctgtctgccggcaaatctcacgtggaactccaggccaagctgaagcaaatcatcctgaagcacaagaccaacctgtctctgattgagcagctcgaggacggcttttcattcttcctgatggcccagttcctgaccagcagcatcctcgtgtgtgtggtgctgtacgagctgaccatggtgttcggctggaacgaggacaccttcaagaccgtgacatacctgcctggcgctatcctgcagctgttcctgttctgttggtacgcccagcagatcaccgaagaggccaggctggtgtccgatcacatctacaacatcccttggtatctggctgaccccaagctgcagaaggacatcctgaccttcatggtcaaggcccagaaacctaccggcgtgaccgccagcaagttctacatggtcaccctgcagaccttccagagaatcagcagcacctcctacagctacttcaccctgctgcagaccatcaaccagcagtaa

SEQ ID NO: 29 - protein, 398 aa, Artificial Sequence
  AgOR28 T25K, P31T, 22a.a del
MARLVLHEVRYVLMAMLYISRGMAKKIQNSTIDLYVYWFLTFIPIASLCVPQFTYLVVDTKSLIDFISVLVPITEILLTNGKMIICNVKRGKIINLINQVQVAWDECAKSEHLEIQTLITTTAKKSKIFVIIYTTSFLLICVEYSSMPLFKLIYHSAVYGKQSNYTIALPYLSRFAYSTESTTSFAWTYFFILIGVYLLALTLSGFDSLFSTLVMHIKMMFKVLKFEIEQLGLDLSAGKSHVELQAKLKQIILKHKTNLSLIEQLEDGFSFFLMAQFLTSSILVCVVLYELTMVFGWNEDTFKTVTYLPGAILQLFLFCWYAQQITEEARLVSDHIYNIPWYLADPKLQKDILTFMVKAQKPTGVTASKFYMVTLQTFQRISSTSYSYFTLLQTINQQ

SEQ ID NO: 30 - DNA, 1197 bp, Artificial Sequence
  AgOR28 T25K, P31T, 22a.a del
atggccagactggtgctgcacgaagtccgctatgtgctgatggccatgctgtacatcagcagaggcatggccaagaagatccagaacagcaccatcgacctgtacgtgtactggttcctgacattcatccctatcgccagcctgtgcgtgccccagttcacctacctggtggtggacaccaagagcctgatcgacttcatcagcgtgctggtgcccatcaccgagatcctgctgaccaacggcaagatgattatctgcaacgtgaagcggggcaagatcatcaacctgatcaaccaggtgcaggtcgcctgggatgagtgtgccaagtctgagcacctggaaatccagacactgatcaccaccaccgccaagaaaagcaagatcttcgtgattatctacaccaccagctttctgctgatctgcgtggaatactccagcatgcccctgttcaagctgatctaccacagcgccgtgtacggcaagcagagcaactacacaatcgccctgccttacctgagcagattcgcctacagcaccgagagcaccacaagcttcgcctggacctacttcttcatcctgatcggcgtgtacctgctggccctgacactgagcggcttcgatagcctgtttagcaccctggtcatgcacatcaagatgatgttcaaggtgctgaagttcgagatcgagcagctgggcctcgatctgtctgccggcaaatctcacgtggaactccaggccaagctgaagcaaatcatcctgaagcacaagaccaacctgtctctgattgagcagctcgaggacggcttttcattcttcctgatggcccagttcctgaccagcagcatcctcgtgtgtgtggtgctgtacgagctgaccatggtgttcggctggaacgaggacaccttcaagaccgtgacatacctgcctggcgctatcctgcagctgttcctgttctgttggtacgcccagcagatcaccgaagaggccaggctggtgtccgatcacatctacaacatcccttggtatctggctgaccccaagctgcagaaggacatcctgaccttcatggtcaaggcccagaaacctaccggcgtgaccgccagcaagttctacatggtcaccctgcagaccttccagagaatcagcagcacctcctacagctacttcaccctgctgcagaccatcaaccagcagtaa

SEQ ID NO: 31 - protein, 387 aa, Artificial Sequence
  AgOR47 L60P
MVVFDPLDDPLKVLPLPLKLLALLGVNKNPSERFRLYAIYAYLCIALFIPKLCLGYETIPQCFRSIAEGMLSFNTTITFIMLPLKMDNLEDLLKNLKRFTEIVIFNEDYEQILIRLNTAIHKFTKYYFIFTNGIVFAMTSSTIAGMFYTYYAKDSEYSAAFPLIMENRLYLIDSHYNLGHCFVHQALMFFALYILLVMFTAKAGTLFGLIRFCSTVLGIIVLKIERLSQIGPVDKYTAELNEIIELHQLAIKCSRQLQNILMEILLAQFTGCVFIWCFMLYYVMISGITAEGIAVVAMLIALSTETFIFCLLGNELTLKGLEISTAMYFTNWYDQPVKLQKMVVPIIQQSQQRIGITAAKFYYIDYNRYGQSLKTAYSFYLLLKDIF

SEQ ID NO: 32 - DNA, 1164 bp, Artificial Sequence
  AgOR47 L60P
atggtggtgttcgaccctctggacgatcccctgaaagtgctgcctctgcctctgaaactgctggccctgctgggcgtgaacaagaaccctagcgagcggttcagactgtacgccatctacgcctacctgtgtatcgccctgttcatccccaagctgtgcctgggctacgagacaatcccgcagtgcttccggtctatcgccgagggcatgctgagcttcaataccaccatcaccttcatcatgctgcccctgaagatggacaacctggaagatctgctgaagaacctgaagcggttcaccgagatcgtgatcttcaacgaggactacgagcagatcctgatccggctgaacaccgccatccacaagttcaccaagtactacttcatcttcaccaacggcatcgtgttcgccatgaccagctctacaatcgccggcatgttctacacctactacgccaaggacagcgagtacagcgccgcctttcctctgatcatggaaaaccggctgtacctgatcgacagccactacaacctgggccactgcttcgtgcaccaggctctgatgttctttgccctgtacatcctgctcgtgatgttcaccgccaaggccggcacactgttcggcctgatcagattctgtagcaccgtgctgggcatcatcgtgctgaagatcgagcggctgtctcagatcggccccgtggataagtataccgccgagctgaacgagatcatcgagctgcaccagctggccatcaagtgcagcagacagctgcagaacatcctgatggaaatcctgctggctcagttcaccggctgcgtgttcatctggtgcttcatgctgtactacgtgatgatcagcggcatcaccgccgagggaattgccgtggtggctatgctgattgccctgtctaccgagactttcatcttctgcctgctgggaaacgagctgaccctgaaaggcctggaaatcagcaccgccatgtacttcacaaattggtacgaccagcctgtgaagctccagaaaatggtggtgcccatcatccagcagtcccagcagagaatcggaatcacagccgccaagttctactacatcgactacaacagatacggccagagcctgaaaaccgcctacagcttctacctgctgctgaaggacatcttctga

SEQ ID NO: 33 - DNA, 30 bp, Artificial Sequence
  Primer
ctacgagacaatcccgcagtgcttccggtc

SEQ ID NO: 34 - DNA, 30 bp, Artificial Sequence
  Primer
gaccggaagcactgcgggattgtctcgtag

SEQ ID NO: 35 - protein, 387 aa, Artificial Sequence
  AgOR47 L71F
MVVFDPLDDPLKVLPLPLKLLALLGVNKNPSERFRLYAIYAYLCIALFIPKLCLGYETILQCFRSIAEGMFSFNTTITFIMLPLKMDNLEDLLKNLKRFTEIVIFNEDYEQILIRLNTAIHKFTKYYFIFTNGIVFAMTSSTIAGMFYTYYAKDSEYSAAFPLIMENRLYLIDSHYNLGHCFVHQALMFFALYILLVMFTAKAGTLFGLIRFCSTVLGIIVLKIERLSQIGPVDKYTAELNEIIELHQLAIKCSRQLQNILMEILLAQFTGCVFIWCFMLYYVMISGITAEGIAVVAMLIALSTETFIFCLLGNELTLKGLEISTAMYFTNWYDQPVKLQKMVVPIIQQSQQRIGITAAKFYYIDYNRYGQSLKTAYSFYLLLKDIF

SEQ ID NO: 36 - DNA, 1164 bp, Artificial Sequence
  AgOR47 L71F
atggtggtgttcgaccctctggacgatcccctgaaagtgctgcctctgcctctgaaactgctggccctgctgggcgtgaacaagaaccctagcgagcggttcagactgtacgccatctacgcctacctgtgtatcgccctgttcatccccaagctgtgcctgggctacgagacaatcctgcagtgcttccggtctatcgccgagggcatgttcagcttcaataccaccatcaccttcatcatgctgcccctgaagatggacaacctggaagatctgctgaagaacctgaagcggttcaccgagatcgtgatcttcaacgaggactacgagcagatcctgatccggctgaacaccgccatccacaagttcaccaagtactacttcatcttcaccaacggcatcgtgttcgccatgaccagctctacaatcgccggcatgttctacacctactacgccaaggacagcgagtacagcgccgcctttcctctgatcatggaaaaccggctgtacctgatcgacagccactacaacctgggccactgcttcgtgcaccaggctctgatgttctttgccctgtacatcctgctcgtgatgttcaccgccaaggccggcacactgttcggcctgatcagattctgtagcaccgtgctgggcatcatcgtgctgaagatcgagcggctgtctcagatcggccccgtggataagtataccgccgagctgaacgagatcatcgagctgcaccagctggccatcaagtgcagcagacagctgcagaacatcctgatggaaatcctgctggctcagttcaccggctgcgtgttcatctggtgcttcatgctgtactacgtgatgatcagcggcatcaccgccgagggaattgccgtggtggctatgctgattgccctgtctaccgagactttcatcttctgcctgctgggaaacgagctgaccctgaaaggcctggaaatcagcaccgccatgtacttcacaaattggtacgaccagcctgtgaagctccagaaaatggtggtgcccatcatccagcagtcccagcagagaatcggaatcacagccgccaagttctactacatcgactacaacagatacggccagagcctgaaaaccgcctacagcttctacctgctgctgaaggacatcttctga

SEQ ID NO: 37 - DNA, 35 bp, Artificial Sequence
  Primer
ctatcgccgagggcatgttcagcttcaataccacc

SEQ ID NO: 38 - DNA, 35 bp, Artificial Sequence
  Primer
ggtggtattgaagctgaacatgccctcggcgatag

SEQ ID NO: 39 - protein, 387 aa, Artificial Sequence
  AgOR47 I134V
MVVFDPLDDPLKVLPLPLKLLALLGVNKNPSERFRLYAIYAYLCIALFIPKLCLGYETILQCFRSIAEGMLSFNTTITFIMLPLKMDNLEDLLKNLKRFTEIVIFNEDYEQILIRLNTAIHKFTKYYFIFTNGVVFAMTSSTIAGMFYTYYAKDSEYSAAFPLIMENRLYLIDSHYNLGHCFVHQALMFFALYILLVMFTAKAGTLFGLIRFCSTVLGIIVLKIERLSQIGPVDKYTAELNEIIELHQLAIKCSRQLQNILMEILLAQFTGCVFIWCFMLYYVMISGITAEGIAVVAMLIALSTETFIFCLLGNELTLKGLEISTAMYFTNWYDQPVKLQKMVVPIIQQSQQRIGITAAKFYYIDYNRYGQSLKTAYSFYLLLKDIF

SEQ ID NO: 40 - DNA, 1164 bp, Artificial Sequence
  AgOR47 I134V
atggtggtgttcgaccctctggacgatcccctgaaagtgctgcctctgcctctgaaactgctggccctgctgggcgtgaacaagaaccctagcgagcggttcagactgtacgccatctacgcctacctgtgtatcgccctgttcatccccaagctgtgcctgggctacgagacaatcctgcagtgcttccggtctatcgccgagggcatgctgagcttcaataccaccatcaccttcatcatgctgcccctgaagatggacaacctggaagatctgctgaagaacctgaagcggttcaccgagatcgtgatcttcaacgaggactacgagcagatcctgatccggctgaacaccgccatccacaagttcaccaagtactacttcatcttcaccaacggcgtcgtgttcgccatgaccagctctacaatcgccggcatgttctacacctactacgccaaggacagcgagtacagcgccgcctttcctctgatcatggaaaaccggctgtacctgatcgacagccactacaacctgggccactgcttcgtgcaccaggctctgatgttctttgccctgtacatcctgctcgtgatgttcaccgccaaggccggcacactgttcggcctgatcagattctgtagcaccgtgctgggcatcatcgtgctgaagatcgagcggctgtctcagatcggccccgtggataagtataccgccgagctgaacgagatcatcgagctgcaccagctggccatcaagtgcagcagacagctgcagaacatcctgatggaaatcctgctggctcagttcaccggctgcgtgttcatctggtgcttcatgctgtactacgtgatgatcagcggcatcaccgccgagggaattgccgtggtggctatgctgattgccctgtctaccgagactttcatcttctgcctgctgggaaacgagctgaccctgaaaggcctggaaatcagcaccgccatgtacttcacaaattggtacgaccagcctgtgaagctccagaaaatggtggtgcccatcatccagcagtcccagcagagaatcggaatcacagccgccaagttctactacatcgactacaacagatacggccagagcctgaaaaccgcctacagcttctacctgctgctgaaggacatcttctga

SEQ ID NO: 41 - DNA, 33 bp, Artificial Sequence
  Primer
catcttcaccaacggcgtcgtgttcgccatgac

SEQ ID NO: 42 - DNA, 34 bp, Artificial Sequence
  Prier
ggtcatggcgaacacgacgccgttggtgaagatg

SEQ ID NO: 43 - protein, 387 aa, Artificial Sequence
  AgOR47 S140G
MVVFDPLDDPLKVLPLPLKLLALLGVNKNPSERFRLYAIYAYLCIALFIPKLCLGYETILQCFRSIAEGMLSFNTTITFIMLPLKMDNLEDLLKNLKRFTEIVIFNEDYEQILIRLNTAIHKFTKYYFIFTNGIVFAMTGSTIAGMFYTYYAKDSEYSAAFPLIMENRLYLIDSHYNLGHCFVHQALMFFALYILLVMFTAKAGTLFGLIRFCSTVLGIIVLKIERLSQIGPVDKYTAELNEIIELHQLAIKCSRQLQNILMEILLAQFTGCVFIWCFMLYYVMISGITAEGIAVVAMLIALSTETFIFCLLGNELTLKGLEISTAMYFTNWYDQPVKLQKMVVPIIQQSQQRIGITAAKFYYIDYNRYGQSLKTAYSFYLLLKDIF

SEQ ID NO: 44 - DNA, 1164 bp, Artificial Sequence
  AgOR47 S140G
atggtggtgttcgaccctctggacgatcccctgaaagtgctgcctctgcctctgaaactgctggccctgctgggcgtgaacaagaaccctagcgagcggttcagactgtacgccatctacgcctacctgtgtatcgccctgttcatccccaagctgtgcctgggctacgagacaatcctgcagtgcttccggtctatcgccgagggcatgctgagcttcaataccaccatcaccttcatcatgctgcccctgaagatggacaacctggaagatctgctgaagaacctgaagcggttcaccgagatcgtgatcttcaacgaggactacgagcagatcctgatccggctgaacaccgccatccacaagttcaccaagtactacttcatcttcaccaacggcatcgtgttcgccatgaccggctctacaatcgccggcatgttctacacctactacgccaaggacagcgagtacagcgccgcctttcctctgatcatggaaaaccggctgtacctgatcgacagccactacaacctgggccactgcttcgtgcaccaggctctgatgttctttgccctgtacatcctgctcgtgatgttcaccgccaaggccggcacactgttcggcctgatcagattctgtagcaccgtgctgggcatcatcgtgctgaagatcgagcggctgtctcagatcggccccgtggataagtataccgccgagctgaacgagatcatcgagctgcaccagctggccatcaagtgcagcagacagctgcagaacatcctgatggaaatcctgctggctcagttcaccggctgcgtgttcatctggtgcttcatgctgtactacgtgatgatcagcggcatcaccgccgagggaattgccgtggtggctatgctgattgccctgtctaccgagactttcatcttctgcctgctgggaaacgagctgaccctgaaaggcctggaaatcagcaccgccatgtacttcacaaattggtacgaccagcctgtgaagctccagaaaatggtggtgcccatcatccagcagtcccagcagagaatcggaatcacagccgccaagttctactacatcgactacaacagatacggccagagcctgaaaaccgcctacagcttctacctgctgctgaaggacatcttctga

SEQ ID NO: 45 - DNA, 32 bp, Artificial Sequence
  Primer
gtgttcgccatgaccggctctacaatcgccgg

SEQ ID NO: 46 - DNA, 32 bp, Artificial Sequence
  Primer
ccggcgattgtagagccggtcatggcgaacac

SEQ ID NO: 47 - protein, 387 aa, Artificial Sequence
  AgOR47 F147L
MVVFDPLDDPLKVLPLPLKLLALLGVNKNPSERFRLYAIYAYLCIALFIPKLCLGYETILQCFRSIAEGMLSFNTTITFIMLPLKMDNLEDLLKNLKRFTEIVIFNEDYEQILIRLNTAIHKFTKYYFIFTNGIVFAMTSSTIAGMLYTYYAKDSEYSAAFPLIMENRLYLIDSHYNLGHCFVHQALMFFALYILLVMFTAKAGTLFGLIRFCSTVLGIIVLKIERLSQIGPVDKYTAELNEIIELHQLAIKCSRQLQNILMEILLAQFTGCVFIWCFMLYYVMISGITAEGIAVVAMLIALSTETFIFCLLGNELTLKGLEISTAMYFTNWYDQPVKLQKMVVPIIQQSQQRIGITAAKFYYIDYNRYGQSLKTAYSFYLLLKDIF

SEQ ID NO: 48 - DNA, 1164 bp, Artificial Sequence
  AgOR47 F147L
atggtggtgttcgaccctctggacgatcccctgaaagtgctgcctctgcctctgaaactgctggccctgctgggcgtgaacaagaaccctagcgagcggttcagactgtacgccatctacgcctacctgtgtatcgccctgttcatccccaagctgtgcctgggctacgagacaatcctgcagtgcttccggtctatcgccgagggcatgctgagcttcaataccaccatcaccttcatcatgctgcccctgaagatggacaacctggaagatctgctgaagaacctgaagcggttcaccgagatcgtgatcttcaacgaggactacgagcagatcctgatccggctgaacaccgccatccacaagttcaccaagtactacttcatcttcaccaacggcatcgtgttcgccatgaccagctctacaatcgccggcatgctctacacctactacgccaaggacagcgagtacagcgccgcctttcctctgatcatggaaaaccggctgtacctgatcgacagccactacaacctgggccactgcttcgtgcaccaggctctgatgttctttgccctgtacatcctgctcgtgatgttcaccgccaaggccggcacactgttcggcctgatcagattctgtagcaccgtgctgggcatcatcgtgctgaagatcgagcggctgtctcagatcggccccgtggataagtataccgccgagctgaacgagatcatcgagctgcaccagctggccatcaagtgcagcagacagctgcagaacatcctgatggaaatcctgctggctcagttcaccggctgcgtgttcatctggtgcttcatgctgtactacgtgatgatcagcggcatcaccgccgagggaattgccgtggtggctatgctgattgccctgtctaccgagactttcatcttctgcctgctgggaaacgagctgaccctgaaaggcctggaaatcagcaccgccatgtacttcacaaattggtacgaccagcctgtgaagctccagaaaatggtggtgcccatcatccagcagtcccagcagagaatcggaatcacagccgccaagttctactacatcgactacaacagatacggccagagcctgaaaaccgcctacagcttctacctgctgctgaaggacatcttctga

SEQ ID NO: 49 - DNA, 32 bp, Artificial Sequence
  Primer
caatcgccggcatgttctacacctactacacc

SEQ ID NO: 50 - DNA, 32 bp, Artificial Sequence
  Primer
ggtgtagtaggtgtagaacatgccggcgattg

SEQ ID NO: 51 - protein, 387 aa, Artificial Sequence
  AgOR47 D5E
MVVFEPLDDPLKVLPLPLKLLALLGVNKNPSERFRLYAIYAYLCIALFIPKLCLGYETILQCFRSIAEGMLSFNTTITFIMLPLKMDNLEDLLKNLKRFTEIVIFNEDYEQILIRLNTAIHKFTKYYFIFTNGIVFAMTSSTIAGMFYTYYAKDSEYSAAFPLIMENRLYLIDSHYNLGHCFVHQALMFFALYILLVMFTAKAGTLFGLIRFCSTVLGIIVLKIERLSQIGPVDKYTAELNEIIELHQLAIKCSRQLQNILMEILLAQFTGCVFIWCFMLYYVMISGITAEGIAVVAMLIALSTETFIFCLLGNELTLKGLEISTAMYFTNWYDQPVKLQKMVVPIIQQSQQRIGITAAKFYYIDYNRYGQSLKTAYSFYLLLKDIF

SEQ ID NO: 52 - DNA, 1164 bp, Artificial Sequence
  AgOR47 D5E
atggtggtgttcgaacctctggacgatcccctgaaagtgctgcctctgcctctgaaactgctggccctgctgggcgtgaacaagaaccctagcgagcggttcagactgtacgccatctacgcctacctgtgtatcgccctgttcatccccaagctgtgcctgggctacgagacaatcctgcagtgcttccggtctatcgccgagggcatgctgagcttcaataccaccatcaccttcatcatgctgcccctgaagatggacaacctggaagatctgctgaagaacctgaagcggttcaccgagatcgtgatcttcaacgaggactacgagcagatcctgatccggctgaacaccgccatccacaagttcaccaagtactacttcatcttcaccaacggcatcgtgttcgccatgaccagctctacaatcgccggcatgttctacacctactacgccaaggacagcgagtacagcgccgcctttcctctgatcatggaaaaccggctgtacctgatcgacagccactacaacctgggccactgcttcgtgcaccaggctctgatgttctttgccctgtacatcctgctcgtgatgttcaccgccaaggccggcacactgttcggcctgatcagattctgtagcaccgtgctgggcatcatcgtgctgaagatcgagcggctgtctcagatcggccccgtggataagtataccgccgagctgaacgagatcatcgagctgcaccagctggccatcaagtgcagcagacagctgcagaacatcctgatggaaatcctgctggctcagttcaccggctgcgtgttcatctggtgcttcatgctgtactacgtgatgatcagcggcatcaccgccgagggaattgccgtggtggctatgctgattgccctgtctaccgagactttcatcttctgcctgctgggaaacgagctgaccctgaaaggcctggaaatcagcaccgccatgtacttcacaaattggtacgaccagcctgtgaagctccagaaaatggtggtgcccatcatccagcagtcccagcagagaatcggaatcacagccgccaagttctactacatcgactacaacagatacggccagagcctgaaaaccgcctacagcttctacctgctgctgaaggacatcttctga

SEQ ID NO: 53 - DNA, 29 bp, Artificial Sequence
  Primer
atggttgtgttcgaaccactggacgaccc

SEQ ID NO: 54 - DNA, 29 bp, Artificial Sequence
  Primer
gggtcgtccagtggttcgaacacaaccat

SEQ ID NO: 55 - protein, 387 aa, Artificial Sequence
  AgOR47 K235Q
MVVFDPLDDPLKVLPLPLKLLALLGVNKNPSERFRLYAIYAYLCIALFIPKLCLGYETILQCFRSIAEGMLSFNTTITFIMLPLKMDNLEDLLKNLKRFTEIVIFNEDYEQILIRLNTAIHKFTKYYFIFTNGIVFAMTSSTIAGMFYTYYAKDSEYSAAFPLIMENRLYLIDSHYNLGHCFVHQALMFFALYILLVMFTAKAGTLFGLIRFCSTVLGIIVLKIERLSQIGPVDQYTAELNEIIELHQLAIKCSRQLQNILMEILLAQFTGCVFIWCFMLYYVMISGITAEGIAVVAMLIALSTETFIFCLLGNELTLKGLEISTAMYFTNWYDQPVKLQKMVVPIIQQSQQRIGITAAKFYYIDYNRYGQSLKTAYSFYLLLKDIF

SEQ ID NO: 56 - DNA, 1164 bp, Artificial Sequence
  AgOR47 K235Q
atggtggtgttcgaccctctggacgatcccctgaaagtgctgcctctgcctctgaaactgctggccctgctgggcgtgaacaagaaccctagcgagcggttcagactgtacgccatctacgcctacctgtgtatcgccctgttcatccccaagctgtgcctgggctacgagacaatcctgcagtgcttccggtctatcgccgagggcatgctgagcttcaataccaccatcaccttcatcatgctgcccctgaagatggacaacctggaagatctgctgaagaacctgaagcggttcaccgagatcgtgatcttcaacgaggactacgagcagatcctgatccggctgaacaccgccatccacaagttcaccaagtactacttcatcttcaccaacggcatcgtgttcgccatgaccagctctacaatcgccggcatgttctacacctactacgccaaggacagcgagtacagcgccgcctttcctctgatcatggaaaaccggctgtacctgatcgacagccactacaacctgggccactgcttcgtgcaccaggctctgatgttctttgccctgtacatcctgctcgtgatgttcaccgccaaggccggcacactgttcggcctgatcagattctgtagcaccgtgctgggcatcatcgtgctgaagatcgagcggctgtctcagatcggccccgtggatcagtataccgccgagctgaacgagatcatcgagctgcaccagctggccatcaagtgcagcagacagctgcagaacatcctgatggaaatcctgctggctcagttcaccggctgcgtgttcatctggtgcttcatgctgtactacgtgatgatcagcggcatcaccgccgagggaattgccgtggtggctatgctgattgccctgtctaccgagactttcatcttctgcctgctgggaaacgagctgaccctgaaaggcctggaaatcagcaccgccatgtacttcacaaattggtacgaccagcctgtgaagctccagaaaatggtggtgcccatcatccagcagtcccagcagagaatcggaatcacagccgccaagttctactacatcgactacaacagatacggccagagcctgaaaaccgcctacagcttctacctgctgctgaaggacatcttctga

SEQ ID NO: 57 - DNA, 34 bp, Artificial Sequence
  Primer
gatcggacccgttgaccagtatactgcagagctg

SEQ ID NO: 58 - DNA, 34 bp, Artificial Sequence
  Primer
cagctctgcagtatactggtcaacgggtccgatc

SEQ ID NO: 59 - protein, 387 aa, Artificial Sequence
  AgOR47 N241S
MVVFDPLDDPLKVLPLPLKLLALLGVNKNPSERFRLYAIYAYLCIALFIPKLCLGYETILQCFRSIAEGMLSFNTTITFIMLPLKMDNLEDLLKNLKRFTEIVIFNEDYEQILIRLNTAIHKFTKYYFIFTNGIVFAMTSSTIAGMFYTYYAKDSEYSAAFPLIMENRLYLIDSHYNLGHCFVHQALMFFALYILLVMFTAKAGTLFGLIRFCSTVLGIIVLKIERLSQIGPVDKYTAELSEIIELHQLAIKCSRQLQNILMEILLAQFTGCVFIWCFMLYYVMISGITAEGIAVVAMLIALSTETFIFCLLGNELTLKGLEISTAMYFTNWYDQPVKLQKMVVPIIQQSQQRIGITAAKFYYIDYNRYGQSLKTAYSFYLLLKDIF

SEQ ID NO: 60 - DNA, 1164 bp, Artificial Sequence
  AgOR47 N241S
atggtggtgttcgaccctctggacgatcccctgaaagtgctgcctctgcctctgaaactgctggccctgctgggcgtgaacaagaaccctagcgagcggttcagactgtacgccatctacgcctacctgtgtatcgccctgttcatccccaagctgtgcctgggctacgagacaatcctgcagtgcttccggtctatcgccgagggcatgctgagcttcaataccaccatcaccttcatcatgctgcccctgaagatggacaacctggaagatctgctgaagaacctgaagcggttcaccgagatcgtgatcttcaacgaggactacgagcagatcctgatccggctgaacaccgccatccacaagttcaccaagtactacttcatcttcaccaacggcatcgtgttcgccatgaccagctctacaatcgccggcatgttctacacctactacgccaaggacagcgagtacagcgccgcctttcctctgatcatggaaaaccggctgtacctgatcgacagccactacaacctgggccactgcttcgtgcaccaggctctgatgttctttgccctgtacatcctgctcgtgatgttcaccgccaaggccggcacactgttcggcctgatcagattctgtagcaccgtgctgggcatcatcgtgctgaagatcgagcggctgtctcagatcggccccgtggataagtataccgccgagctgagtgagatcatcgagctgcaccagctggccatcaagtgcagcagacagctgcagaacatcctgatggaaatcctgctggctcagttcaccggctgcgtgttcatctggtgcttcatgctgtactacgtgatgatcagcggcatcaccgccgagggaattgccgtggtggctatgctgattgccctgtctaccgagactttcatcttctgcctgctgggaaacgagctgaccctgaaaggcctggaaatcagcaccgccatgtacttcacaaattggtacgaccagcctgtgaagctccagaaaatggtggtgcccatcatccagcagtcccagcagagaatcggaatcacagccgccaagttctactacatcgactacaacagatacggccagagcctgaaaaccgcctacagcttctacctgctgctgaaggacatcttctga

SEQ ID NO: 61 - DNA, 37 bp, Artificial Sequence
  Primer
gtatactgcagagctgagtgaaattatcgaacttcac

SEQ ID NO: 62 - DNA, 37 bp, Artificial Sequence
  Primer
gtgaagttcgataatttcactcagctctgcagtatac

SEQ ID NO: 63 - protein, 387 aa, Artificial Sequence
  AgOR47 M138I
MVVFDPLDDPLKVLPLPLKLLALLGVNKNPSERFRLYAIYAYLCIALFIPKLCLGYETILQCFRSIAEGMLSFNTTITFIMLPLKMDNLEDLLKNLKRFTEIVIFNEDYEQILIRLNTAIHKFTKYYFIFTNGIVFAITSSTIAGMFYTYYAKDSEYSAAFPLIMENRLYLIDSHYNLGHCFVHQALMFFALYILLVMFTAKAGTLFGLIRFCSTVLGIIVLKIERLSQIGPVDKYTAELNEIIELHQLAIKCSRQLQNILMEILLAQFTGCVFIWCFMLYYVMISGITAEGIAVVAMLIALSTETFIFCLLGNELTLKGLEISTAMYFTNWYDQPVKLQKMVVPIIQQSQQRIGITAAKFYYIDYNRYGQSLKTAYSFYLLLKDIF

SEQ ID NO: 64 - DNA, 1164 bp, Artificial Sequence
  AgOR47 M138I
atggtggtgttcgaccctctggacgatcccctgaaagtgctgcctctgcctctgaaactgctggccctgctgggcgtgaacaagaaccctagcgagcggttcagactgtacgccatctacgcctacctgtgtatcgccctgttcatccccaagctgtgcctgggctacgagacaatcctgcagtgcttccggtctatcgccgagggcatgctgagcttcaataccaccatcaccttcatcatgctgcccctgaagatggacaacctggaagatctgctgaagaacctgaagcggttcaccgagatcgtgatcttcaacgaggactacgagcagatcctgatccggctgaacaccgccatccacaagttcaccaagtactacttcatcttcaccaacggcatcgtgttcgccatcaccagctctacaatcgccggcatgttctacacctactacgccaaggacagcgagtacagcgccgcctttcctctgatcatggaaaaccggctgtacctgatcgacagccactacaacctgggccactgcttcgtgcaccaggctctgatgttctttgccctgtacatcctgctcgtgatgttcaccgccaaggccggcacactgttcggcctgatcagattctgtagcaccgtgctgggcatcatcgtgctgaagatcgagcggctgtctcagatcggccccgtggataagtataccgccgagctgaacgagatcatcgagctgcaccagctggccatcaagtgcagcagacagctgcagaacatcctgatggaaatcctgctggctcagttcaccggctgcgtgttcatctggtgcttcatgctgtactacgtgatgatcagcggcatcaccgccgagggaattgccgtggtggctatgctgattgccctgtctaccgagactttcatcttctgcctgctgggaaacgagctgaccctgaaaggcctggaaatcagcaccgccatgtacttcacaaattggtacgaccagcctgtgaagctccagaaaatggtggtgcccatcatccagcagtcccagcagagaatcggaatcacagccgccaagttctactacatcgactacaacagatacggccagagcctgaaaaccgcctacagcttctacctgctgctgaaggacatcttctga

SEQ ID NO: 65 - DNA, 33 bp, Artificial Sequence
  Primer
ggcgtcgtgttcgccatcaccggctctacaatc

SEQ ID NO: 66 - DNA, 33 bp, Artificial Sequence
  Primer
gattgtagagccggtgatggcgaacacgacgcc

SEQ ID NO: 67 - protein, 387 aa, Artificial Sequence
  AgOR47 A152T
MVVFDPLDDPLKVLPLPLKLLALLGVNKNPSERFRLYAIYAYLCIALFIPKLCLGYETILQCFRSIAEGMLSFNTTITFIMLPLKMDNLEDLLKNLKRFTEIVIFNEDYEQILIRLNTAIHKFTKYYFIFTNGIVFAMTSSTIAGMFYTYYTKDSEYSAAFPLIMENRLYLIDSHYNLGHCFVHQALMFFALYILLVMFTAKAGTLFGLIRFCSTVLGIIVLKIERLSQIGPVDKYTAELNEIIELHQLAIKCSRQLQNILMEILLAQFTGCVFIWCFMLYYVMISGITAEGIAVVAMLIALSTETFIFCLLGNELTLKGLEISTAMYFTNWYDQPVKLQKMVVPIIQQSQQRIGITAAKFYYIDYNRYGQSLKTAYSFYLLLKDIF

SEQ ID NO: 68 - DNA, 1164 bp, Artificial Sequence
  AgOR47 A152T
atggtggtgttcgaccctctggacgatcccctgaaagtgctgcctctgcctctgaaactgctggccctgctgggcgtgaacaagaaccctagcgagcggttcagactgtacgccatctacgcctacctgtgtatcgccctgttcatccccaagctgtgcctgggctacgagacaatcctgcagtgcttccggtctatcgccgagggcatgctgagcttcaataccaccatcaccttcatcatgctgcccctgaagatggacaacctggaagatctgctgaagaacctgaagcggttcaccgagatcgtgatcttcaacgaggactacgagcagatcctgatccggctgaacaccgccatccacaagttcaccaagtactacttcatcttcaccaacggcatcgtgttcgccatgaccagctctacaatcgccggcatgttctacacctactacaccaaggacagcgagtacagcgccgcctttcctctgatcatggaaaaccggctgtacctgatcgacagccactacaacctgggccactgcttcgtgcaccaggctctgatgttctttgccctgtacatcctgctcgtgatgttcaccgccaaggccggcacactgttcggcctgatcagattctgtagcaccgtgctgggcatcatcgtgctgaagatcgagcggctgtctcagatcggccccgtggataagtataccgccgagctgaacgagatcatcgagctgcaccagctggccatcaagtgcagcagacagctgcagaacatcctgatggaaatcctgctggctcagttcaccggctgcgtgttcatctggtgcttcatgctgtactacgtgatgatcagcggcatcaccgccgagggaattgccgtggtggctatgctgattgccctgtctaccgagactttcatcttctgcctgctgggaaacgagctgaccctgaaaggcctggaaatcagcaccgccatgtacttcacaaattggtacgaccagcctgtgaagctccagaaaatggtggtgcccatcatccagcagtcccagcagagaatcggaatcacagccgccaagttctactacatcgactacaacagatacggccagagcctgaaaaccgcctacagcttctacctgctgctgaaggacatcttctga

SEQ ID NO: 69 - DNA, 42 bp, Artificial Sequence
  Primer
ggaatgttttacacctactacacgaaagattcggaatattcc

SEQ ID NO: 70 - DNA, 42 bp, Artificial Sequence
  Primer
ggaatattccgaatctttcgtgtagtaggtgtaaaacattcc

SEQ ID NO: 71 - protein, 387 aa, Artificial Sequence
  AgOR47 L60P L71F A152T
MVVFDPLDDPLKVLPLPLKLLALLGVNKNPSERFRLYAIYAYLCIALFIPKLCLGYETIPQCFRSIAEGMLSFNTTITFIMLPLKMDNLEDLLKNLKRFTEIVIFNEDYEQILIRLNTAIHKFTKYYFIFTNGIVFAMTSSTIAGMFYTYYTKDSEYSAAFPLIMENRLYLIDSHYNLGHCFVHQALMFFALYILLVMFTAKAGTLFGLIRFCSTVLGIIVLKIERLSQIGPVDKYTAELNEIIELHQLAIKCSRQLQNILMEILLAQFTGCVFIWCFMLYYVMISGITAEGIAVVAMLIALSTETFIFCLLGNELTLKGLEISTAMYFTNWYDQPVKLQKMVVPIIQQSQQRIGITAAKFYYIDYNRYGQSLKTAYSFYLLLKDIF

SEQ ID NO: 72 - DNA, 1164 bp, Artificial Sequence
  AgOR47 L60P L71F A152T
atggtggtgttcgaccctctggacgatcccctgaaagtgctgcctctgcctctgaaactgctggccctgctgggcgtgaacaagaaccctagcgagcggttcagactgtacgccatctacgcctacctgtgtatcgccctgttcatccccaagctgtgcctgggctacgagacaatcccgcagtgcttccggtctatcgccgagggcatgctgagcttcaataccaccatcaccttcatcatgctgcccctgaagatggacaacctggaagatctgctgaagaacctgaagcggttcaccgagatcgtgatcttcaacgaggactacgagcagatcctgatccggctgaacaccgccatccacaagttcaccaagtactacttcatcttcaccaacggcatcgtgttcgccatgaccagctctacaatcgccggcatgttctacacctactacaccaaggacagcgagtacagcgccgcctttcctctgatcatggaaaaccggctgtacctgatcgacagccactacaacctgggccactgcttcgtgcaccaggctctgatgttctttgccctgtacatcctgctcgtgatgttcaccgccaaggccggcacactgttcggcctgatcagattctgtagcaccgtgctgggcatcatcgtgctgaagatcgagcggctgtctcagatcggccccgtggataagtataccgccgagctgaacgagatcatcgagctgcaccagctggccatcaagtgcagcagacagctgcagaacatcctgatggaaatcctgctggctcagttcaccggctgcgtgttcatctggtgcttcatgctgtactacgtgatgatcagcggcatcaccgccgagggaattgccgtggtggctatgctgattgccctgtctaccgagactttcatcttctgcctgctgggaaacgagctgaccctgaaaggcctggaaatcagcaccgccatgtacttcacaaattggtacgaccagcctgtgaagctccagaaaatggtggtgcccatcatccagcagtcccagcagagaatcggaatcacagccgccaagttctactacatcgactacaacagatacggccagagcctgaaaaccgcctacagcttctacctgctgctgaaggacatcttctga

SEQ ID NO: 73 - protein, 387 aa, Artificial Sequence
  AgOR47 L60P L71F I134V A152T
MVVFDPLDDPLKVLPLPLKLLALLGVNKNPSERFRLYAIYAYLCIALFIPKLCLGYETILQCFRSIAEGMLSFNTTITFIMLPLKMDNLEDLLKNLKRFTEIVIFNEDYEQILIRLNTAIHKFTKYYFIFTNGIVFAITSSTIAGMFYTYYTKDSEYSAAFPLIMENRLYLIDSHYNLGHCFVHQALMFFALYILLVMFTAKAGTLFGLIRFCSTVLGIIVLKIERLSQIGPVDKYTAELNEIIELHQLAIKCSRQLQNILMEILLAQFTGCVFIWCFMLYYVMISGITAEGIAVVAMLIALSTETFIFCLLGNELTLKGLEISTAMYFTNWYDQPVKLQKMVVPIIQQSQQRIGITAAKFYYIDYNRYGQSLKTAYSFYLLLKDIF

SEQ ID NO: 74 - DNA, 1164 bp, Artificial Sequence
  AgOR47 L60P L71F I134V A152T
atggtggtgttcgaccctctggacgatcccctgaaagtgctgcctctgcctctgaaactgctggccctgctgggcgtgaacaagaaccctagcgagcggttcagactgtacgccatctacgcctacctgtgtatcgccctgttcatccccaagctgtgcctgggctacgagacaatcctgcagtgcttccggtctatcgccgagggcatgctgagcttcaataccaccatcaccttcatcatgctgcccctgaagatggacaacctggaagatctgctgaagaacctgaagcggttcaccgagatcgtgatcttcaacgaggactacgagcagatcctgatccggctgaacaccgccatccacaagttcaccaagtactacttcatcttcaccaacggcatcgtgttcgccatcaccagctctacaatcgccggcatgttctacacctactacaccaaggacagcgagtacagcgccgcctttcctctgatcatggaaaaccggctgtacctgatcgacagccactacaacctgggccactgcttcgtgcaccaggctctgatgttctttgccctgtacatcctgctcgtgatgttcaccgccaaggccggcacactgttcggcctgatcagattctgtagcaccgtgctgggcatcatcgtgctgaagatcgagcggctgtctcagatcggccccgtggataagtataccgccgagctgaacgagatcatcgagctgcaccagctggccatcaagtgcagcagacagctgcagaacatcctgatggaaatcctgctggctcagttcaccggctgcgtgttcatctggtgcttcatgctgtactacgtgatgatcagcggcatcaccgccgagggaattgccgtggtggctatgctgattgccctgtctaccgagactttcatcttctgcctgctgggaaacgagctgaccctgaaaggcctggaaatcagcaccgccatgtacttcacaaattggtacgaccagcctgtgaagctccagaaaatggtggtgcccatcatccagcagtcccagcagagaatcggaatcacagccgccaagttctactacatcgactacaacagatacggccagagcctgaaaaccgcctacagcttctacctgctgctgaaggacatcttctga

SEQ ID NO: 75 - protein, 387 aa, Artificial Sequence
  AgOR47 L60P L71F I134V S140G A152T
MVVFDPLDDPLKVLPLPLKLLALLGVNKNPSERFRLYAIYAYLCIALFIPKLCLGYETIPQCFRSIAEGMLSFNTTITFIMLPLKMDNLEDLLKNLKRFTEIVIFNEDYEQILIRLNTAIHKFTKYYFIFTNGIVFAITSSTIAGMFYTYYTKDSEYSAAFPLIMENRLYLIDSHYNLGHCFVHQALMFFALYILLVMFTAKAGTLFGLIRFCSTVLGIIVLKIERLSQIGPVDKYTAELNEIIELHQLAIKCSRQLQNILMEILLAQFTGCVFIWCFMLYYVMISGITAEGIAVVAMLIALSTETFIFCLLGNELTLKGLEISTAMYFTNWYDQPVKLQKMVVPIIQQSQQRIGITAAKFYYIDYNRYGQSLKTAYSFYLLLKDIF

SEQ ID NO: 76 - DNA, 1164 bp, Artificial Sequence
  AgOR47 L60P L71F I134V S140G A152T
atggtggtgttcgaccctctggacgatcccctgaaagtgctgcctctgcctctgaaactgctggccctgctgggcgtgaacaagaaccctagcgagcggttcagactgtacgccatctacgcctacctgtgtatcgccctgttcatccccaagctgtgcctgggctacgagacaatcccgcagtgcttccggtctatcgccgagggcatgctgagcttcaataccaccatcaccttcatcatgctgcccctgaagatggacaacctggaagatctgctgaagaacctgaagcggttcaccgagatcgtgatcttcaacgaggactacgagcagatcctgatccggctgaacaccgccatccacaagttcaccaagtactacttcatcttcaccaacggcatcgtgttcgccatcaccagctctacaatcgccggcatgttctacacctactacaccaaggacagcgagtacagcgccgcctttcctctgatcatggaaaaccggctgtacctgatcgacagccactacaacctgggccactgcttcgtgcaccaggctctgatgttctttgccctgtacatcctgctcgtgatgttcaccgccaaggccggcacactgttcggcctgatcagattctgtagcaccgtgctgggcatcatcgtgctgaagatcgagcggctgtctcagatcggccccgtggataagtataccgccgagctgaacgagatcatcgagctgcaccagctggccatcaagtgcagcagacagctgcagaacatcctgatggaaatcctgctggctcagttcaccggctgcgtgttcatctggtgcttcatgctgtactacgtgatgatcagcggcatcaccgccgagggaattgccgtggtggctatgctgattgccctgtctaccgagactttcatcttctgcctgctgggaaacgagctgaccctgaaaggcctggaaatcagcaccgccatgtacttcacaaattggtacgaccagcctgtgaagctccagaaaatggtggtgcccatcatccagcagtcccagcagagaatcggaatcacagccgccaagttctactacatcgactacaacagatacggccagagcctgaaaaccgcctacagcttctacctgctgctgaaggacatcttctga

SEQ ID NO: 77 - protein, 387 aa, Artificial Sequence
  AgOR47 L60P L71F I134V M138I S140G F147L A152T
MVVFDPLDDPLKVLPLPLKLLALLGVNKNPSERFRLYAIYAYLCIALFIPKLCLGYETIPQCFRSIAEGMFSFNTTITFIMLPLKMDNLEDLLKNLKRFTEIVIFNEDYEQILIRLNTAIHKFTKYYFIFTNGVVFAITGSTIAGMLYTYYTKDSEYSAAFPLIMENRLYLIDSHYNLGHCFVHQALMFFALYILLVMFTAKAGTLFGLIRFCSTVLGIIVLKIERLSQIGPVDKYTAELNEIIELHQLAIKCSRQLQNILMEILLAQFTGCVFIWCFMLYYVMISGITAEGIAVVAMLIALSTETFIFCLLGNELTLKGLEISTAMYFTNWYDQPVKLQKMVVPIIQQSQQRIGITAAKFYYIDYNRYGQSLKTAYSFYLLLKDIF

SEQ ID NO: 78 - DNA, 1164 bp, Artificial Sequence
  AgOR47 L60P L71F I134V M138I S140G F147L A152T
atggtggtgttcgaccctctggacgatcccctgaaagtgctgcctctgcctctgaaactgctggccctgctgggcgtgaacaagaaccctagcgagcggttcagactgtacgccatctacgcctacctgtgtatcgccctgttcatccccaagctgtgcctgggctacgagacaatcccgcagtgcttccggtctatcgccgagggcatgttcagcttcaataccaccatcaccttcatcatgctgcccctgaagatggacaacctggaagatctgctgaagaacctgaagcggttcaccgagatcgtgatcttcaacgaggactacgagcagatcctgatccggctgaacaccgccatccacaagttcaccaagtactacttcatcttcaccaacggcgtcgtgttcgccatcaccggctctacaatcgccggcatgctctacacctactacaccaaggacagcgagtacagcgccgcctttcctctgatcatggaaaaccggctgtacctgatcgacagccactacaacctgggccactgcttcgtgcaccaggctctgatgttctttgccctgtacatcctgctcgtgatgttcaccgccaaggccggcacactgttcggcctgatcagattctgtagcaccgtgctgggcatcatcgtgctgaagatcgagcggctgtctcagatcggccccgtggataagtataccgccgagctgaacgagatcatcgagctgcaccagctggccatcaagtgcagcagacagctgcagaacatcctgatggaaatcctgctggctcagttcaccggctgcgtgttcatctggtgcttcatgctgtactacgtgatgatcagcggcatcaccgccgagggaattgccgtggtggctatgctgattgccctgtctaccgagactttcatcttctgcctgctgggaaacgagctgaccctgaaaggcctggaaatcagcaccgccatgtacttcacaaattggtacgaccagcctgtgaagctccagaaaatggtggtgcccatcatccagcagtcccagcagagaatcggaatcacagccgccaagttctactacatcgactacaacagatacggccagagcctgaaaaccgcctacagcttctacctgctgctgaaggacatcttctga

SEQ ID NO: 79 - protein, 387 aa, Artificial Sequence
  AgOR47 L60P L71F I134V M138I S140G F147L
MVVFDPLDDPLKVLPLPLKLLALLGVNKNPSERFRLYAIYAYLCIALFIPKLCLGYETIPQCFRSIAEGMFSFNTTITFIMLPLKMDNLEDLLKNLKRFTEIVIFNEDYEQILIRLNTAIHKFTKYYFIFTNGVVFAITGSTIAGMLYTYYAKDSEYSAAFPLIMENRLYLIDSHYNLGHCFVHQALMFFALYILLVMFTAKAGTLFGLIRFCSTVLGIIVLKIERLSQIGPVDKYTAELNEIIELHQLAIKCSRQLQNILMEILLAQFTGCVFIWCFMLYYVMISGITAEGIAVVAMLIALSTETFIFCLLGNELTLKGLEISTAMYFTNWYDQPVKLQKMVVPIIQQSQQRIGITAAKFYYIDYNRYGQSLKTAYSFYLLLKDIF

SEQ ID NO: 80 - DNA, 1164 bp, Artificial Sequence
  AgOR47 L60P L71F I134V M138I S140G F147L
atggtggtgttcgaccctctggacgatcccctgaaagtgctgcctctgcctctgaaactgctggccctgctgggcgtgaacaagaaccctagcgagcggttcagactgtacgccatctacgcctacctgtgtatcgccctgttcatccccaagctgtgcctgggctacgagacaatcccgcagtgcttccggtctatcgccgagggcatgttcagcttcaataccaccatcaccttcatcatgctgcccctgaagatggacaacctggaagatctgctgaagaacctgaagcggttcaccgagatcgtgatcttcaacgaggactacgagcagatcctgatccggctgaacaccgccatccacaagttcaccaagtactacttcatcttcaccaacggcgtcgtgttcgccatcaccggctctacaatcgccggcatgctctacacctactacgccaaggacagcgagtacagcgccgcctttcctctgatcatggaaaaccggctgtacctgatcgacagccactacaacctgggccactgcttcgtgcaccaggctctgatgttctttgccctgtacatcctgctcgtgatgttcaccgccaaggccggcacactgttcggcctgatcagattctgtagcaccgtgctgggcatcatcgtgctgaagatcgagcggctgtctcagatcggccccgtggataagtataccgccgagctgaacgagatcatcgagctgcaccagctggccatcaagtgcagcagacagctgcagaacatcctgatggaaatcctgctggctcagttcaccggctgcgtgttcatctggtgcttcatgctgtactacgtgatgatcagcggcatcaccgccgagggaattgccgtggtggctatgctgattgccctgtctaccgagactttcatcttctgcctgctgggaaacgagctgaccctgaaaggcctggaaatcagcaccgccatgtacttcacaaattggtacgaccagcctgtgaagctccagaaaatggtggtgcccatcatccagcagtcccagcagagaatcggaatcacagccgccaagttctactacatcgactacaacagatacggccagagcctgaaaaccgcctacagcttctacctgctgctgaaggacatcttctga

SEQ ID NO: 81 - protein, 405 aa, Artificial Sequence
  AgOR6 mut
MVRLSFEETLRNTNLMLLMMGIPPCEEPYPPGVLPSLKRNAGFIASFLLLAYTTIGELIYLKQMFERDVTFLEVTFQAPCIGYCTIGVLKMVILARGRNTIAELVGLFRAKWTAAIVTGEHWAVCEDTMRPAIRVTSVTALANVVMGIAFTILPIAEMIYTYHYTGRWNRQLAFNIWWPFDVLGGAKYYWFVYPLYVVIGFTGIIIHMAFDCLFCILAAHLCMQFRILAHNFGHVVEVANGAGEGIGDSGSTSRLQDAIRIHQELIGCSVFMQNVFGNALFINFLGSSIIICIQAFMITTVSGYMLVKFVLFMLCFLIELLMLCAYGEDIVESSLGVIDAAYGCEWYREGSMAFHRSVLQIIHRSQQPVILTAWKIWPIQMSTFSQILQASWSYFTLLKTVYGNK

SEQ ID NO: 82 - DNA, 1218 bp, Artificial Sequence
  AgOR6 mut
atggtacgtctaagctttgaagaaacgctacgaaacaccaacctgatgctactgatgatgggcattccaccgtgcgaggagccgtacccgccgggcgtactgccgtcgctcaaacgcaacgcgggctttatcgcgtccttcctgctgctcgcctacaccacgatcggtgagctgatctatctgaagcagatgtttgagcgggacgttaccttcctggaggtaacctttcaagcgccctgcatcgggtactgcaccatcggtgtgctgaagatggtcatactggcccggggaaggaacacgatcgccgagctggtcggtttgtttcgcgcaaagtggaccgcggcgattgtaaccggtgagcattgggcggtgtgcgaggacacaatgcggcccgccattcgggtcacctcggtaacggcgctcgcgaacgtcgtgatggggatagcgttcaccatcctgccgatcgcggagatgatctacacctatcactacaccggccggtggaaccgtcagcttgccttcaacatctggtggccgttcgatgtgctgggaggcgcgaagtactactggttcgtctatccactgtacgtggtgattgggttcacgggcatcatcatccatatggcgttcgactgtttgttctgcatactggcggcccatctctgtatgcagtttcgcatcctggcgcacaactttggccatgtggtagaggttgccaatggtgctggtgaaggtataggtgacagtggcagtacgagtcggctacaggatgcgatcagaatccatcaggagttgattggctgcagcgtgttcatgcagaacgtgtttggcaatgcgctgtttattaacttcctcggcagctccatcataatctgcatccaggcgtttatgataacgacggttagcggatatatgctggtaaagtttgtcctcttcatgctgtgctttctgatcgagctgctgatgctgtgtgcgtacggtgaggatattgtggaatcgagccttggggtgattgatgccgcttacggttgcgaatggtaccgggaagggtcgatggcgttccatcgatccgtgctgcaaattatacaccgcagccagcagcccgtcatactgacggcgtggaaaatctggcccatccaaatgagtaccttcagtcagatcctgcaagcttcctggtcctactttaccctcctgaagaccgtctacgggaataagtaa

SEQ ID NO: 83 - protein, 387 aa, Artificial Sequence
  AgOR15 mut
MNFLRQEQPAGMPHISIKLLRVFGVTNHSEERFRIVPVMLAYFFFIVVPKCFFGYPDLEITIIGTAELIFQTNSFCGMFLLFLNRRKLAEFIQHARSFSQTVIRASPPAVVQHLTTQHDMIHKITRIFCIVVMFAAHFYALAPFLSTLYTFYGTVRNKNATMHYTLQMEENFYGLQTRTSATHYLIFGIVMTPTAYLCAFTGTVKTLTICNITTYCTLYFQLVQLKLRTVTQDNTFRQELKSVIKMHQDALNCASLVESITSLALLQQLLLCVLIWSSMLLYFTVSGFNVNFMNLFVLFVFDTTETFAYCYLGEKLSYESARVAHTVYESGWETQTTDIQKDLQLILVRAQSPVGITAGKFYYMNMEQFGIIVKTTYSFFVILRDQI

SEQ ID NO: 84 - DNA, 1164 bp, Artificial Sequence
  AgOR15 mut
atgaacttcctaagacaggagcaaccggctggcatgcctcatatctccatcaagctgctccgggtatttggcgttaccaatcattcagaggaacgctttcgtatcgtgccggttatgctggcctactttttcttcatagtagtgcccaagtgtttcttcggatatcccgaccttgagataacgatcattggcaccgctgagctgattttccaaaccaactccttttgtggaatgtttctgttgtttctgaacagacgcaaactggctgagttcattcaacatgctagaagtttctcccaaacggttatccgtgcgtcacctcccgcggtggtccagcatttgacgacccagcacgacatgatccacaagataaccagaatcttctgcatcgtagtgatgtttgcagctcacttctacgcattagctccttttctttctacgctttacacgttttacggtacggtacggaacaaaaacgcaaccatgcactacacgctgcaaatggaggaaaacttctacggactacagactcgcacctcggctacgcactacctgatcttcggtatcgtcatgacgcctaccgcgtatctctgtgccttcaccggcacggtgaagactctaaccatctgtaatattactacctactgtaccctttactttcaattggtacaactgaagctacgaaccgtcacgcaggacaacacattccgtcaagagttgaagtcggtgatcaagatgcatcaggatgcacttaactgtgcaagtctggtagaatctatcacgtcactagcgctattacagcaactgcttctatgcgtattgatctggagctcaatgttgctttacttcaccgtatcgggattcaatgtgaactttatgaatcttttcgtactgttcgtgttcgacacaacggaaacctttgcctactgttatcttggggaaaagctatcgtacgagagtgctcgtgtagcacataccgtttacgaaagtggctgggaaactcaaaccaccgacatacagaaagatcttcagctaattcttgtccgtgctcaaagtccagttggcatcactgctggcaagttttactacatgaacatggaacagtttggcattatagtaaaaactacctactcgttctttgtgatattgcgggatcagatttaa

SEQ ID NO: 85 - protein, 406 aa, Aedes aegypti
MTQSLEFDQTFGFIAKVLQMIGYPSCLAPYPTTFASRLKSSAGFVVCFLMLTYCVFGQIINIGLLMMGHRQTDQVVEEVAIQVSSTGFCIIGLAKMYSLSYNRAILSWLIADFRVKWNAGELTDKDRSIRDGTLRPTVAITTVAALGNIIMVSAFNFQPVVEMIYGRVVTGEWVKLFPYVIWFPFNSTHGAIYYLVYLFEVYSGVIVAVGNVGFNCIFCLLTSHLSMQLKLLCSWIEDMVEVEDEKGVQSKKKLYRIVRYHQDLIRGRNALQSMFSTTLFLNFSASSVLMCMQLYLITTAGITLMVKFTLFMLCILMEIFILCYYGEEILANSSSIAAGAFNSNWYQSKVSQQNPRFGKNLIPIIQQGQRPMVLTAWKFWPITIRTFSAILQTSWSYFTLLKTVMH

SEQ ID NO: 86 - DNA, 1221 bp, Aedes aegypti
atgactcaatcccttgagtttgaccaaacctttggcttcatcgccaaggtcttgcaaatgatcggttatccaagctgtttagcaccgtacccaacgaccttcgccagtcgactcaagtccagtgccggtttcgtggtatgcttcctcatgttgacctattgcgttttcggtcagatcatcaacatcggcctgctgatgatgggtcaccgccagacggatcaggtcgtcgaagaggtcgccatccaggtcagcagcacaggcttttgcatcatcggactggcgaagatgtacagtttgtcgtacaaccgggccattctgagctggctcattgcggacttcagagtcaagtggaatgccggggaactcacagataaggaccgttccatacgggacgggacgttacgtccaacggtggccattacgactgtagcggcattagggaacatcataatggtgtcggcgttcaactttcaaccggtggtggagatgatctacggtcgggtggttaccggagaatgggtcaagctatttccgtacgtgatttggttccctttcaattcgactcacggggcgatctactatctggtgtacttgtttgaggtttattcgggagttatagtggccgttggaaacgtggggttcaactgtatcttctgtttgctgacttcacacttgtcgatgcagttaaagctgttgtgcagttggatcgaggatatggttgaagttgaggacgagaagggggtgcaatcgaagaagaagctctacaggattgtgcggtatcatcaggacttgatcagaggaaggaatgcgttacaatcaatgttcagcacaacgctgttcctgaacttctccgcaagttctgttctgatgtgcatgcagctttacctcataactaccgcaggcattactctgatggtcaagtttactcttttcatgctttgtattttgatggagattttcattctctgctactacggtgaagagattctcgctaatagttcatcgattgccgctggagcgttcaactcgaattggtaccagtcgaaggtgagccaacagaatcctcgttttggcaaaaatttgattccgattatccagcaagggcagaggcccatggttctgacggcgtggaagttttggcccataaccattcggacgttcagcgccatattgcaaacatcatggtcctattttaccttgctgaaaactgtaatgcattag

SEQ ID NO: 87 - protein, 344 aa, Artificial Sequence
  rho-myc-mOlfr256_17
MNGTEGPNFYVPFSNKTGVVEQKLISEEDLEFMEVDSNSSSGSFILMGVSDHPHLEIIFFAVILASYLLTLVGNLTIILLSRLDARLHTPMYFFLSNLSSLDLAFTTSSVPQMLKNLWGPDKTISYGGCVTQLYVFLWLGATECILLVVMAFDRYVAVCRPLHYMTVMNPRLCWGLAAISWLGGLGNSVIQSTFTLQLPFCGHRKVDNFLCEVPAMIKLACGDTSLNEAVLNGVCTFFTVVPVSVILVSYCFIAQAVMKIRSVEGRRKAFNTCVSHLVVVFLFYGSAIYGYLLPAKSSNQSQGKFISLFYSVVTPMVNPLIYTLRNKEVKGALGRLLGKGRGAS

SEQ ID NO: 88 - protein, 374 aa, Mus musculus
MARSLTWGCCPWCLTEEEKTAARIDQEINRILLEQKKQEREELKLLLLGPGESGKSTFIKQMRIIHGVGYSEEDRRAFRLLIYQNIFVSMQAMIDAMDRLQIPFSRPDSKQHASLVMTQDPYKVSTFEKPYAVAMQYLWRDAGIRACYERRREFHLLDSAVYYLSHLERISEDSYIPTAQDVLRSRMPTTGINEYCFSVKKTKLRIVDVGGQRSERRKWIHCFENVIALIYLASLSEYDQCLEENDQENRMEESLALFSTILELPWFKSTSVILFLNKTDILEDKIHTSHLATYFPSFQGPRRDAEAAKSFILDMYARVYASCAEPQDGGRKGSRARRFFAHFTCATDTQSVRSVFKDVRDSVLARYLKQYELL

SEQ ID NO: 89 - protein, 227 aa, Mus musculus
MCKSVTTGEWKKVFYEKMEEVKPADSWDFIIDPNLKHNVLAPGWKQYLELHASGRFHCSWCWHTWQSPHVVILFHMYLDKAQRAGSVRMRVFKQLCYECGTARLDESSMLEENIESLVDNLITSLREQCYGERGGHYRIHVASRQDNRRHRGEFCEACQEGIVHWKPSEKLLEEEATTYTFSRAPSPTKPQAETGSGCNFCSIPWCLFWATVLMLIIYLQFSFRTSV

SEQ ID NO: 90 - DNA, 48 bp, Artificial Sequence
  Primer
gccagcctgtgcgtgccccagttcacctacctggtggtggacaccaag

SEQ ID NO: 91 - DNA, 46 bp, Artificial Sequence
  Primer
caccaggtaggtgaactggggcacgcacaggctggcgatagggatg

SEQ ID NO: 92 - protein, 480 aa, Artificial Sequence
  Dm(NT-TM4)AaORCO
MTTSMQPSKYTGLVADLMPNIRAMKYSGLFMHNFTGGSAFMKKVYSSVHLVFLLMQFTFILVNMALNAEEVNELSGNTITTLFFTHCITKFIYLAVNQKNFYRTLNIWNQVNTHPLFAESDARYHSIALAKMRKLFFLVMLTTVASATAWTTITFFGDSVKMVVDHETNSSIPVEIPRLPIKSFYPWNASHGMFYMISFAFQIYYVLFSMIHSNLCDVMFCSWLIFACEQLQHLKNIMKPLMEFSATLDTVVPNSGELFKAGSAEQPKEQEPLPPVTPPQGENMLDMDLRGIYSNRTDFTTTFRPTAGMTFNGGVGPNGLTKKQEMLVRSAIKYWVERHKHIVRLVTAIGDAYGVALLLHMLTTTITLTLLAYQATKIHAVDTYAASVVGYLLYSLGQVFMLCIFGNRLIEESSSVMEAAYSCHWYDGSEEAKTFVQIVCQQCQKAMSISGAKFFTVSLDLFASVLGAMVTYFMVLVQLK

SEQ ID NO: 93 - DNA, 1443 bp, Artificial Sequence
  Dm(NT-TM4)AaORCO
atgacaacctcgatgcagccgagcaagtacacgggcctggtcgccgacctgatgcccaacatccgggcgatgaagtactccggcctgttcatgcacaacttcacgggcggcagtgccttcatgaagaaggtgtactcctccgtgcacctggtgttcctcctcatgcagttcaccttcatcctggtcaacatggccctgaacgccgaggaggtcaacgagctgtcgggcaacacgatcacgaccctcttcttcacccactgcatcacgaagtttatctacctggctgttaaccagaagaatttctacagaacattgaatatatggaaccaggtgaacacgcatcccttgttcgccgagtcggatgctcgttaccattcgatcgcactggcgaagatgaggaagctgttctttctggtgatgctgaccacagtcgcctcggccaccgcctggaccacgatcaccttctttggcgacagcgtaaaaatggtggtggaccatgagacgaactccagcatcccggtggagataccccggctgccgattaagtccttctacccgtggaacgccagccacggcatgttctacatgatcagctttgcctttcagatctactacgtgctcttctcgatgatccactccaatctatgcgacgtgatgttctgctcttggctgatattcgcctgcgagcagctgcagcacttgaagaatatcatgaagcctttgatggaattcagcgccacgctggacaccgtcgtgccaaacagtggggaactgttcaaggctggcagtgcagagcagccgaaggaacaggagccattgccaccagtcacgccgccccagggtgaaaacatgttggacatggatcttcgagggatatatagcaacaggaccgacttcacgaccaccttccggccaactgctggaatgacgttcaacggcggggtcgggccaaatgggttgaccaagaaacaggaaatgctggtacgaagcgccatcaagtactgggtagagagacacaagcatatcgttagactcgtaactgcaattggagacgcctatggtgtagctttgctgctacatatgttgactactactattacgttaactttgctcgcttaccaagcaacaaagatacatgcagtagatacatacgcagcatcagtagtaggttatttgctatattctttaggacaagtctttatgctctgtatatttggaaatcgtctcattgaagagagctcatcagtgatggaagcagcttattcttgtcactggtatgatggatcagaggaggccaaaacatttgtacagattgtttgccagcagtgtcagaaagcgatgtcgatttcaggggcaaagttcttcactgtatctttggatctctttgcttcggtgttgggagctatggttacctacttcatggtgttggtgcaactgaagtga

SEQ ID NO: 94 - DNA, 34 bp, Artificial Sequence
  Primer
cccgaccttgagataacgatcattggcaccgctg

SEQ ID NO: 95 - DNA, 34 bp, Artificial Sequence
  Primer
cagcggtgccaatgatcgttatctcaaggtcggg

SEQ ID NO: 96 - DNA, 32 bp, Artificial Sequence
  Primer
cccaaacggttatccgtgcgtcacctcccgcg

SEQ ID NO: 97 - DNA, 32 bp, Artificial Sequence
  Primer
cgcgggaggtgacgcacggataaccgtttggg

SEQ ID NO: 98 - DNA, 33 bp, Artificial Sequence
  Primer
cctcccgcggtggtccagcatttgacgacccag

SEQ ID NO: 99 - DNA, 33 bp, Artificial Sequence
  Primer
ctgggtcgtcaaatgctggaccaccgcgggagg

SEQ ID NO: 100 - DNA, 33 bp, Artificial Sequence
  Primer
cagactcgcacctcggctacgcactacctgatc

SEQ ID NO: 101 - DNA, 33 bp, Artificial Sequence
  Primer
gatcaggtagtgcgtagccgaggtgcgagtctg

SEQ ID NO: 102 - DNA, 34 bp, Artificial Sequence
  Primer
ctacctgatcttcggtatcgtcatgacgcctacc

SEQ ID NO: 103 - DNA, 34 bp, Artificial Sequence
  Primer
ggtaggcgtcatgacgataccgaagatcaggtag

SEQ ID NO: 104 - DNA, 33 bp, Artificial Sequence
  Primer
cgtgtagcacataccgtttacgaaagtggctgg

SEQ ID NO: 105 - DNA, 33 bp, Artificial Sequence
  Primer
ccagccactttcgtaaacggtatgtgctacacg

SEQ ID NO: 106 - DNA, 32 bp, Artificial Sequence
  Primer
gggtcaagctatttccgtacgtgatttggttc

SEQ ID NO: 107 - DNA, 32 bp, Artificial Sequence
  Primer
gaaccaaatcacgtacggaaatagcttgaccc

SEQ ID NO: 108 - protein, 387 aa, Artificial Sequence
  AgOR47 EL60P-L71F-I134V-S140G-F147L
MVVFDPLDDPLKVLPLPLKLLALLGVNKNPSERFRLYAIYAYLCIALFIPKLCLGYETIPQCFRSIAEGMFSFNTTITFIMLPLKMDNLEDLLKNLKRFTEIVIFNEDYEQILIRLNTAIHKFTKYYFIFTNGVVFAMTGSTIAGMLYTYYAKDSEYSAAFPLIMENRLYLIDSHYNLGHCFVHQALMFFALYILLVMFTAKAGTLFGLIRFCSTVLGIIVLKIERLSQIGPVDKYTAELNEIIELHQLAIKCSRQLQNILMEILLAQFTGCVFIWCFMLYYVMISGITAEGIAVVAMLIALSTETFIFCLLGNELTLKGLEISTAMYFTNWYDQPVKLQKMVVPIIQQSQQRIGITAAKFYYIDYNRYGQSLKTAYSFYLLLKDIF

SEQ ID NO: 109 - DNA, 1164 bp, Artificial Sequence
  AgOR47 EL60P-L71F-I134V-S140G-F147L
atggtggtgttcgaccctctggacgatcccctgaaagtgctgcctctgcctctgaaactgctggccctgctgggcgtgaacaagaaccctagcgagcggttcagactgtacgccatctacgcctacctgtgtatcgccctgttcatccccaagctgtgcctgggctacgagacaatcccgcagtgcttccggtctatcgccgagggcatgttcagcttcaataccaccatcaccttcatcatgctgcccctgaagatggacaacctggaagatctgctgaagaacctgaagcggttcaccgagatcgtgatcttcaacgaggactacgagcagatcctgatccggctgaacaccgccatccacaagttcaccaagtactacttcatcttcaccaacggcgtcgtgttcgccatgaccggctctacaatcgccggcatgctctacacctactacgccaaggacagcgagtacagcgccgcctttcctctgatcatggaaaaccggctgtacctgatcgacagccactacaacctgggccactgcttcgtgcaccaggctctgatgttctttgccctgtacatcctgctcgtgatgttcaccgccaaggccggcacactgttcggcctgatcagattctgtagcaccgtgctgggcatcatcgtgctgaagatcgagcggctgtctcagatcggccccgtggataagtataccgccgagctgaacgagatcatcgagctgcaccagctggccatcaagtgcagcagacagctgcagaacatcctgatggaaatcctgctggctcagttcaccggctgcgtgttcatctggtgcttcatgctgtactacgtgatgatcagcggcatcaccgccgagggaattgccgtggtggctatgctgattgccctgtctaccgagactttcatcttctgcctgctgggaaacgagctgaccctgaaaggcctggaaatcagcaccgccatgtacttcacaaattggtacgaccagcctgtgaagctccagaaaatggtggtgcccatcatccagcagtcccagcagagaatcggaatcacagccgccaagttctactacatcgactacaacagatacggccagagcctgaaaaccgcctacagcttctacctgctgctgaaggacatcttctga